European Patent Application EP 4 733 313 A2, published April 29, 2026. Title: MACROCYCLIC MODULATORS OF DISEASE ASSOCIATED PROTEIN MISFOLDING AND AGGREGATION. Applicant: ResQ Biotech P.C. Application EP. The sequence listing filed with the application follows.

SEQUENCE LISTING (515 sequences)

SEQ ID NO: 1 - protein, 5 aa, synthetic construct
  REGION 1..5: note = SOD1C5-1 peptide selected for its ability to rescue themisfolding and modulate the aggregation of SOD1
TASWW

SEQ ID NO: 2 - protein, 5 aa, synthetic construct
  REGION 1..5: note = SOD1C5-2 peptide selected for its ability to rescue themisfolding and modulate the aggregation of SOD1
TASFW

SEQ ID NO: 3 - protein, 5 aa, synthetic construct
  REGION 1..5: note = SOD1C5-3 peptide selected for its ability to rescue themisfolding and modulate the aggregation of SOD1
TSSFW

SEQ ID NO: 4 - protein, 5 aa, synthetic construct
  REGION 1..5: note = SOD1C5-4 peptide selected for its ability to rescue themisfolding and modulate the aggregation of SOD1
TWSVW

SEQ ID NO: 5 - protein, 5 aa, synthetic construct
  REGION 1..5: note = SOD1C5-5 peptide selected for its ability to rescue themisfolding and modulate the aggregation of SOD1
TASHW

SEQ ID NO: 6 - protein, 5 aa, synthetic construct
  REGION 1..5: note = SOD1C5-6 peptide selected for its ability to rescue themisfolding and modulate the aggregation of SOD1
TFSMW

SEQ ID NO: 7 - protein, 5 aa, synthetic construct
  REGION 1..5: note = SOD1C5-7 peptide selected for its ability to rescue themisfolding and modulate the aggregation of SOD1
TASMW

SEQ ID NO: 8 - protein, 5 aa, synthetic construct
  REGION 1..5: note = SOD1C5-9 peptide selected for its ability to rescue themisfolding and modulate the aggregation of SOD1
TVSFW

SEQ ID NO: 9 - protein, 5 aa, synthetic construct
  REGION 1..5: note = SOD1C5-11 peptide selected for its ability to rescue themisfolding and modulate the aggregation of SOD1
TLSFW

SEQ ID NO: 10 - protein, 5 aa, synthetic construct
  REGION 1..5: note = SOD1C5-13 peptide selected for its ability to rescue themisfolding and modulate the aggregation of SOD1
TASRW

SEQ ID NO: 11 - protein, 5 aa, synthetic construct
  REGION 1..5: note = SOD1C5-14 peptide selected for its ability to rescue themisfolding and modulate the aggregation of SOD1
TASSW

SEQ ID NO: 12 - protein, 5 aa, synthetic construct
  REGION 1..5: note = SOD1C5-18 peptide selected for its ability to rescue themisfolding and modulate the aggregation of SOD1
TASLW

SEQ ID NO: 13 - protein, 5 aa, synthetic construct
  REGION 1..5: note = SOD1C5-20 peptide selected for its ability to rescue themisfolding and modulate the aggregation of SOD1
TSSSW

SEQ ID NO: 14 - protein, 5 aa, synthetic construct
  REGION 1..5: note = SOD1C5-23 peptide selected for its ability to rescue themisfolding and modulate the aggregation of SOD1
TGSVW

SEQ ID NO: 15 - protein, 5 aa, synthetic construct
  REGION 1..5: note = SOD1C5-25 peptide selected for its ability to rescue themisfolding and modulate the aggregation of SOD1
TWSLW

SEQ ID NO: 16 - protein, 5 aa, synthetic construct
  REGION 1..5: note = SOD1C5-27 peptide selected for its ability to rescue themisfolding and modulate the aggregation of SOD1
TLSMW

SEQ ID NO: 17 - protein, 5 aa, synthetic construct
  REGION 1..5: note = SOD1C5-31 peptide selected for its ability to rescue themisfolding and modulate the aggregation of SOD1
TWSAW

SEQ ID NO: 18 - protein, 5 aa, synthetic construct
  REGION 1..5: note = SOD1C5-32 peptide selected for its ability to rescue themisfolding and modulate the aggregation of SOD1
TGSWW

SEQ ID NO: 19 - protein, 5 aa, synthetic construct
  REGION 1..5: note = SOD1C5-33 peptide selected for its ability to rescue themisfolding and modulate the aggregation of SOD1
TRSVW

SEQ ID NO: 20 - protein, 5 aa, synthetic construct
  REGION 1..5: note = SOD1C5-39 peptide selected for its ability to rescue themisfolding and modulate the aggregation of SOD1
TSSLW

SEQ ID NO: 21 - protein, 5 aa, synthetic construct
  REGION 1..5: note = SOD1C5-44 peptide selected for its ability to rescue themisfolding and modulate the aggregation of SOD1
TASTW

SEQ ID NO: 22 - protein, 5 aa, synthetic construct
  REGION 1..5: note = SOD1C5-46 peptide selected for its ability to rescue themisfolding and modulate the aggregation of SOD1
TSSVW

SEQ ID NO: 23 - protein, 5 aa, synthetic construct
  REGION 1..5: note = SOD1C5-53 peptide selected for its ability to rescue themisfolding and modulate the aggregation of SOD1
TTSWW

SEQ ID NO: 24 - protein, 5 aa, synthetic construct
  REGION 1..5: note = SOD1C5-65 peptide selected for its ability to rescue themisfolding and modulate the aggregation of SOD1
TASVW

SEQ ID NO: 25 - protein, 5 aa, synthetic construct
  REGION 1..5: note = SOD1C5-74 peptide selected for its ability to rescue themisfolding and modulate the aggregation of SOD1
TCSWW

SEQ ID NO: 26 - protein, 5 aa, synthetic construct
  REGION 1..5: note = SOD1C5-75 peptide selected for its ability to rescue themisfolding and modulate the aggregation of SOD1
TPSFW

SEQ ID NO: 27 - protein, 5 aa, synthetic construct
  REGION 1..5: note = SOD1C5-76 peptide selected for its ability to rescue themisfolding and modulate the aggregation of SOD1
TTSFW

SEQ ID NO: 28 - protein, 5 aa, synthetic construct
  REGION 1..5: note = SOD1C5-80 peptide selected for its ability to rescue themisfolding and modulate the aggregation of SOD1
TFSTW

SEQ ID NO: 29 - protein, 5 aa, synthetic construct
  REGION 1..5: note = SOD1C5-82 peptide selected for its ability to rescue themisfolding and modulate the aggregation of SOD1
TSSMW

SEQ ID NO: 30 - protein, 5 aa, synthetic construct
  REGION 1..5: note = SOD1C5-89 peptide selected for its ability to rescue themisfolding and modulate the aggregation of SOD1
TVSWW

SEQ ID NO: 31 - protein, 5 aa, synthetic construct
  REGION 1..5: note = SOD1C5-93 peptide selected for its ability to rescue themisfolding and modulate the aggregation of SOD1
TDSWW

SEQ ID NO: 32 - protein, 5 aa, synthetic construct
  REGION 1..5: note = SOD1C5-105 peptide selected for its ability to rescue themisfolding and modulate the aggregation of SOD1
TSSWW

SEQ ID NO: 33 - protein, 5 aa, synthetic construct
  REGION 1..5: note = SOD1C5-106 peptide selected for its ability to rescue themisfolding and modulate the aggregation of SOD1
TRSWW

SEQ ID NO: 34 - protein, 5 aa, synthetic construct
  REGION 1..5: note = SOD1C5-109 peptide selected for its ability to rescue themisfolding and modulate the aggregation of SOD1
TWSMW

SEQ ID NO: 35 - protein, 5 aa, synthetic construct
  REGION 1..5: note = SOD1C5-116 peptide selected for its ability to rescue themisfolding and modulate the aggregation of SOD1
TASGW

SEQ ID NO: 36 - protein, 5 aa, synthetic construct
  REGION 1..5: note = SOD1C5-130 peptide selected for its ability to rescue themisfolding and modulate the aggregation of SOD1
TPSWW

SEQ ID NO: 37 - protein, 5 aa, synthetic construct
  REGION 1..5: note = SOD1C5-135 peptide selected for its ability to rescue themisfolding and modulate the aggregation of SOD1
TRSFW

SEQ ID NO: 38 - protein, 5 aa, synthetic construct
  REGION 1..5: note = SOD1C5-140 peptide selected for its ability to rescue themisfolding and modulate the aggregation of SOD1
TSSYW

SEQ ID NO: 39 - protein, 5 aa, synthetic construct
  REGION 1..5: note = SOD1C5-143 peptide selected for its ability to rescue themisfolding and modulate the aggregation of SOD1
TLSVW

SEQ ID NO: 40 - protein, 5 aa, synthetic construct
  REGION 1..5: note = SOD1C5-148 peptide selected for its ability to rescue themisfolding and modulate the aggregation of SOD1
TYSWW

SEQ ID NO: 41 - protein, 5 aa, synthetic construct
  REGION 1..5: note = SOD1C5-160 peptide selected for its ability to rescue themisfolding and modulate the aggregation of SOD1
TFSVW

SEQ ID NO: 42 - protein, 5 aa, synthetic construct
  REGION 1..5: note = SOD1C5-164 peptide selected for its ability to rescue themisfolding and modulate the aggregation of SOD1
TCSVW

SEQ ID NO: 43 - protein, 5 aa, synthetic construct
  REGION 1..5: note = SOD1C5-167 peptide selected for its ability to rescue themisfolding and modulate the aggregation of SOD1
TVSSW

SEQ ID NO: 44 - protein, 5 aa, synthetic construct
  REGION 1..5: note = SOD1C5-168 peptide selected for its ability to rescue themisfolding and modulate the aggregation of SOD1
TRSHW

SEQ ID NO: 45 - protein, 5 aa, synthetic construct
  REGION 1..5: note = SOD1C5-182 peptide selected for its ability to rescue themisfolding and modulate the aggregation of SOD1
TGSAW

SEQ ID NO: 46 - protein, 5 aa, synthetic construct
  REGION 1..5: note = SOD1C5-188 peptide selected for its ability to rescue themisfolding and modulate the aggregation of SOD1
TASYW

SEQ ID NO: 47 - protein, 5 aa, synthetic construct
  REGION 1..5: note = C5-2 peptide selected for its ability to modulate theaggregation of the -amyloid peptide
TTYAR

SEQ ID NO: 48 - protein, 5 aa, synthetic construct
  REGION 1..5: note = C5-3 peptide selected for its ability to modulate theaggregation of the -amyloid peptide
TTVDR

SEQ ID NO: 49 - protein, 5 aa, synthetic construct
  REGION 1..5: note = C5-5 peptide selected for its ability to modulate theaggregation of the -amyloid peptide
TTTWR

SEQ ID NO: 50 - protein, 5 aa, synthetic construct
  REGION 1..5: note = C5-7 peptide selected for its ability to modulate theaggregation of the -amyloid peptide
TTLHR

SEQ ID NO: 51 - protein, 5 aa, synthetic construct
  REGION 1..5: note = C5-8 peptide selected for its ability to modulate theaggregation of the -amyloid peptide
TTFAR

SEQ ID NO: 52 - protein, 5 aa, synthetic construct
  REGION 1..5: note = C5-9 peptide selected for its ability to modulate theaggregation of the -amyloid peptide
TVLDR

SEQ ID NO: 53 - protein, 5 aa, synthetic construct
  REGION 1..5: note = C5-12 peptide selected for its ability to modulate theaggregation of the -amyloid peptide
TTWAR

SEQ ID NO: 54 - protein, 5 aa, synthetic construct
  REGION 1..5: note = C5-13 peptide selected for its ability to modulate theaggregation of the -amyloid peptide
TALDR

SEQ ID NO: 55 - protein, 5 aa, synthetic construct
  REGION 1..5: note = C5-15 peptide selected for its ability to modulate theaggregation of the -amyloid peptide
TANVR

SEQ ID NO: 56 - protein, 5 aa, synthetic construct
  REGION 1..5: note = C5-17 peptide selected for its ability to modulate theaggregation of the -amyloid peptide
TTTAR

SEQ ID NO: 57 - protein, 5 aa, synthetic construct
  REGION 1..5: note = C5-18 peptide selected for its ability to modulate theaggregation of the -amyloid peptide
TTIAR

SEQ ID NO: 58 - protein, 5 aa, synthetic construct
  REGION 1..5: note = C5-19 peptide selected for its ability to modulate theaggregation of the -amyloid peptide
TVWDR

SEQ ID NO: 59 - protein, 5 aa, synthetic construct
  REGION 1..5: note = C5-20 peptide selected for its ability to modulate theaggregation of the -amyloid peptide
TTISR

SEQ ID NO: 60 - protein, 5 aa, synthetic construct
  REGION 1..5: note = C5-21 peptide selected for its ability to modulate theaggregation of the -amyloid peptide
TTWCR

SEQ ID NO: 61 - protein, 5 aa, synthetic construct
  REGION 1..5: note = C5-22 peptide selected for its ability to modulate theaggregation of the -amyloid peptide
TVLWR

SEQ ID NO: 62 - protein, 5 aa, synthetic construct
  REGION 1..5: note = C5-25 peptide selected for its ability to modulate theaggregation of the -amyloid peptide
TTLAR

SEQ ID NO: 63 - protein, 5 aa, synthetic construct
  REGION 1..5: note = C5-26 peptide selected for its ability to modulate theaggregation of the -amyloid peptide
TAWCR

SEQ ID NO: 64 - protein, 5 aa, synthetic construct
  REGION 1..5: note = C5-27 peptide selected for its ability to modulate theaggregation of the -amyloid peptide
TTSAR

SEQ ID NO: 65 - protein, 5 aa, synthetic construct
  REGION 1..5: note = C5-29 peptide selected for its ability to modulate theaggregation of the -amyloid peptide
TTLER

SEQ ID NO: 66 - protein, 5 aa, synthetic construct
  REGION 1..5: note = C5-30 peptide selected for its ability to modulate theaggregation of the -amyloid peptide
TSTAR

SEQ ID NO: 67 - protein, 5 aa, synthetic construct
  REGION 1..5: note = C5-35 peptide selected for its ability to modulate theaggregation of the -amyloid peptide
TVRDR

SEQ ID NO: 68 - protein, 5 aa, synthetic construct
  REGION 1..5: note = C5-41 peptide selected for its ability to modulate theaggregation of the -amyloid peptide
TGWAR

SEQ ID NO: 69 - protein, 5 aa, synthetic construct
  REGION 1..5: note = C5-44 peptide selected for its ability to modulate theaggregation of the -amyloid peptide
TAWAR

SEQ ID NO: 70 - protein, 5 aa, synthetic construct
  REGION 1..5: note = C5-45 peptide selected for its ability to modulate theaggregation of the -amyloid peptide
TTWVR

SEQ ID NO: 71 - protein, 5 aa, synthetic construct
  REGION 1..5: note = C5-46 peptide selected for its ability to modulate theaggregation of the -amyloid peptide
TLLWR

SEQ ID NO: 72 - protein, 5 aa, synthetic construct
  REGION 1..5: note = C5-47 peptide selected for its ability to modulate theaggregation of the -amyloid peptide
TTIDR

SEQ ID NO: 73 - protein, 5 aa, synthetic construct
  REGION 1..5: note = C5-50 peptide selected for its ability to modulate theaggregation of the -amyloid peptide
TALAR

SEQ ID NO: 74 - protein, 5 aa, synthetic construct
  REGION 1..5: note = C5-51 peptide selected for its ability to modulate theaggregation of the -amyloid peptide
TSVDR

SEQ ID NO: 75 - protein, 5 aa, synthetic construct
  REGION 1..5: note = C5-53 peptide selected for its ability to modulate theaggregation of the -amyloid peptide
TTVWR

SEQ ID NO: 76 - protein, 5 aa, synthetic construct
  REGION 1..5: note = C5-66 peptide selected for its ability to modulate theaggregation of the -amyloid peptide
TTHWR

SEQ ID NO: 77 - protein, 5 aa, synthetic construct
  REGION 1..5: note = C5-67 peptide selected for its ability to modulate theaggregation of the -amyloid peptide
TARDR

SEQ ID NO: 78 - protein, 5 aa, synthetic construct
  REGION 1..5: note = C5-73 peptide selected for its ability to modulate theaggregation of the -amyloid peptide
TTRDR

SEQ ID NO: 79 - protein, 5 aa, synthetic construct
  REGION 1..5: note = C5-80 peptide selected for its ability to modulate theaggregation of the -amyloid peptide
TSVHR

SEQ ID NO: 80 - protein, 5 aa, synthetic construct
  REGION 1..5: note = C5-82 peptide selected for its ability to modulate theaggregation of the -amyloid peptide
TAVWR

SEQ ID NO: 81 - protein, 5 aa, synthetic construct
  REGION 1..5: note = C5-83 peptide selected for its ability to modulate theaggregation of the -amyloid peptide
TTGCR

SEQ ID NO: 82 - protein, 5 aa, synthetic construct
  REGION 1..5: note = C5-89 peptide selected for its ability to modulate theaggregation of the -amyloid peptide
TATDR

SEQ ID NO: 83 - protein, 5 aa, synthetic construct
  REGION 1..5: note = C5-94 peptide selected for its ability to modulate theaggregation of the -amyloid peptide
TVLFR

SEQ ID NO: 84 - protein, 5 aa, synthetic construct
  REGION 1..5: note = C5-102 peptide selected for its ability to modulate theaggregation of the -amyloid peptide
TTYNR

SEQ ID NO: 85 - protein, 5 aa, synthetic construct
  REGION 1..5: note = C5-105 peptide selected for its ability to modulate theaggregation of the -amyloid peptide
TVRWR

SEQ ID NO: 86 - protein, 5 aa, synthetic construct
  REGION 1..5: note = C5-116 peptide selected for its ability to modulate theaggregation of the -amyloid peptide
TAFDR

SEQ ID NO: 87 - protein, 5 aa, synthetic construct
  REGION 1..5: note = C5-117 peptide selected for its ability to modulate theaggregation of the -amyloid peptide
TTRCR

SEQ ID NO: 88 - protein, 5 aa, synthetic construct
  REGION 1..5: note = C5-118 peptide selected for its ability to modulate theaggregation of the -amyloid peptide
TTFWR

SEQ ID NO: 89 - protein, 5 aa, synthetic construct
  REGION 1..5: note = C5-121 peptide selected for its ability to modulate theaggregation of the -amyloid peptide
TIKDR

SEQ ID NO: 90 - protein, 5 aa, synthetic construct
  REGION 1..5: note = C5-123 peptide selected for its ability to modulate theaggregation of the -amyloid peptide
TTVHR

SEQ ID NO: 91 - protein, 5 aa, synthetic construct
  REGION 1..5: note = C5-126 peptide selected for its ability to modulate theaggregation of the -amyloid peptide
TTLLR

SEQ ID NO: 92 - protein, 5 aa, synthetic construct
  REGION 1..5: note = C5-129 peptide selected for its ability to modulate theaggregation of the -amyloid peptide
TTLFR

SEQ ID NO: 93 - protein, 5 aa, synthetic construct
  REGION 1..5: note = C5-130 peptide selected for its ability to modulate theaggregation of the -amyloid peptide
TAYHR

SEQ ID NO: 94 - protein, 5 aa, synthetic construct
  REGION 1..5: note = C5-136 peptide selected for its ability to modulate theaggregation of the -amyloid peptide
TALHR

SEQ ID NO: 95 - protein, 5 aa, synthetic construct
  REGION 1..5: note = C5-139 peptide selected for its ability to modulate theaggregation of the -amyloid peptide
TTSPR

SEQ ID NO: 96 - protein, 5 aa, synthetic construct
  REGION 1..5: note = C5-146 peptide selected for its ability to modulate theaggregation of the -amyloid peptide
TTWSR

SEQ ID NO: 97 - protein, 5 aa, synthetic construct
  REGION 1..5: note = C5-147 peptide selected for its ability to modulate theaggregation of the -amyloid peptide
TAMHR

SEQ ID NO: 98 - protein, 5 aa, synthetic construct
  REGION 1..5: note = C5-155 peptide selected for its ability to modulate theaggregation of the -amyloid peptide
TSLDR

SEQ ID NO: 99 - protein, 5 aa, synthetic construct
  REGION 1..5: note = C5-158 peptide selected for its ability to modulate theaggregation of the -amyloid peptide
TTGAR

SEQ ID NO: 100 - protein, 5 aa, synthetic construct
  REGION 1..5: note = C5-162 peptide selected for its ability to modulate theaggregation of the -amyloid peptide
TSVWR

SEQ ID NO: 101 - protein, 5 aa, synthetic construct
  REGION 1..5: note = C5-173 peptide selected for its ability to modulate theaggregation of the -amyloid peptide
TTHAR

SEQ ID NO: 102 - protein, 5 aa, synthetic construct
  REGION 1..5: note = C5-176 peptide selected for its ability to modulate theaggregation of the -amyloid peptide
TAGWR

SEQ ID NO: 103 - protein, 5 aa, synthetic construct
  REGION 1..5: note = C5-177 peptide selected for its ability to modulate theaggregation of the -amyloid peptide
TATAR

SEQ ID NO: 104 - protein, 5 aa, synthetic construct
  REGION 1..5: note = C5-184 peptide selected for its ability to modulate theaggregation of the -amyloid peptide
TVLAR

SEQ ID NO: 105 - protein, 5 aa, synthetic construct
  REGION 1..5: note = C5-185 peptide selected for its ability to modulate theaggregation of the -amyloid peptide
TTFNR

SEQ ID NO: 106 - protein, 5 aa, synthetic construct
  REGION 1..5: note = C5-188 peptide selected for its ability to modulate theaggregation of the -amyloid peptide
TGMRR

SEQ ID NO: 107 - protein, 5 aa, synthetic construct
  REGION 1..5: note = C5-189 peptide selected for its ability to modulate theaggregation of the -amyloid peptide
TTVAR

SEQ ID NO: 108 - protein, 5 aa, synthetic construct
  REGION 1..5: note = AC5-190 peptide selected for its ability to modulate theaggregation of the -amyloid peptide
TLCLR

SEQ ID NO: 109 - protein, 5 aa, synthetic construct
  REGION 1..5: note = C5-192 peptide selected for its ability to modulate theaggregation of the -amyloid peptide
TGLAR

SEQ ID NO: 110 - protein, 5 aa, synthetic construct
  REGION 1..5: note = C5-198 peptide selected for its ability to modulate theaggregation of the -amyloid peptide
TSWCR

SEQ ID NO: 111 - protein, 5 aa, synthetic construct
  REGION 1..5: note = C5-209 peptide selected for its ability to modulate theaggregation of the -amyloid peptide
TTRAR

SEQ ID NO: 112 - protein, 5 aa, synthetic construct
  REGION 1..5: note = C5-215 peptide selected for its ability to modulate theaggregation of the -amyloid peptide
TTPWR

SEQ ID NO: 113 - protein, 5 aa, synthetic construct
  REGION 1..5: note = C5-218 peptide selected for its ability to modulate theaggregation of the -amyloid peptide
TVLHR

SEQ ID NO: 114 - protein, 5 aa, synthetic construct
  REGION 1..5: note = C5-223 peptide selected for its ability to modulate theaggregation of the -amyloid peptide
TGLDR

SEQ ID NO: 115 - protein, 5 aa, synthetic construct
  REGION 1..5: note = C5-230 peptide selected for its ability to modulate theaggregation of the -amyloid peptide
TTSDR

SEQ ID NO: 116 - protein, 5 aa, synthetic construct
  REGION 1..5: note = C5-239 peptide selected for its ability to modulate theaggregation of the -amyloid peptide
TTMHR

SEQ ID NO: 117 - protein, 5 aa, synthetic construct
  REGION 1..5: note = C5-242 peptide selected for its ability to modulate theaggregation of the -amyloid peptide
TTSTR

SEQ ID NO: 118 - protein, 5 aa, synthetic construct
  REGION 1..5: note = C5-244 peptide selected for its ability to modulate theaggregation of the -amyloid peptide
TTRVR

SEQ ID NO: 119 - protein, 5 aa, synthetic construct
  REGION 1..5: note = C5-245 peptide selected for its ability to modulate theaggregation of the -amyloid peptide
TTRFR

SEQ ID NO: 120 - protein, 5 aa, synthetic construct
  REGION 1..5: note = C5-248 peptide selected for its ability to modulate theaggregation of the -amyloid peptide
TTTHR

SEQ ID NO: 121 - protein, 5 aa, synthetic construct
  REGION 1..5: note = C5-250 peptide selected for its ability to modulate theaggregation of the -amyloid peptide
THAWR

SEQ ID NO: 122 - protein, 5 aa, synthetic construct
  REGION 1..5: note = C5-252 peptide selected for its ability to modulate theaggregation of the -amyloid peptide
TVIWR

SEQ ID NO: 123 - protein, 5 aa, synthetic construct
  REGION 1..5: note = C5-253 peptide selected for its ability to modulate theaggregation of the -amyloid peptide
TTWFR

SEQ ID NO: 124 - protein, 5 aa, synthetic construct
  REGION 1..5: note = C5-255 peptide selected for its ability to modulate theaggregation of the -amyloid peptide
TTSRR

SEQ ID NO: 125 - protein, 5 aa, synthetic construct
  REGION 1..5: note = C5-258 peptide selected for its ability to modulate theaggregation of the -amyloid peptide
TTSCR

SEQ ID NO: 126 - protein, 5 aa, synthetic construct
  REGION 1..5: note = C5-260 peptide selected for its ability to modulate theaggregation of the -amyloid peptide
TTWTR

SEQ ID NO: 127 - protein, 5 aa, synthetic construct
  REGION 1..5: note = C5-262 peptide selected for its ability to modulate theaggregation of the -amyloid peptide
TTSSR

SEQ ID NO: 128 - protein, 5 aa, synthetic construct
  REGION 1..5: note = C5-263 peptide selected for its ability to modulate theaggregation of the -amyloid peptide
THLAR

SEQ ID NO: 129 - protein, 5 aa, synthetic construct
  REGION 1..5: note = C5-264 peptide selected for its ability to modulate theaggregation of the -amyloid peptide
TSGAR

SEQ ID NO: 130 - protein, 5 aa, synthetic construct
  REGION 1..5: note = C5-266 peptide selected for its ability to modulate theaggregation of the -amyloid peptide
TTLRR

SEQ ID NO: 131 - protein, 5 aa, synthetic construct
  REGION 1..5: note = C5-270 peptide selected for its ability to modulate theaggregation of the -amyloid peptide
TATWR

SEQ ID NO: 132 - protein, 5 aa, synthetic construct
  REGION 1..5: note = C5-272 peptide selected for its ability to modulate theaggregation of the -amyloid peptide
TCMWR

SEQ ID NO: 133 - protein, 5 aa, synthetic construct
  REGION 1..5: note = C5-275 peptide selected for its ability to modulate theaggregation of the -amyloid peptide
TAHVR

SEQ ID NO: 134 - protein, 5 aa, synthetic construct
  REGION 1..5: note = C5-276 peptide selected for its ability to modulate theaggregation of the -amyloid peptide
TSWAR

SEQ ID NO: 135 - protein, 5 aa, synthetic construct
  REGION 1..5: note = C5-278 peptide selected for its ability to modulate theaggregation of the -amyloid peptide
TTWLR

SEQ ID NO: 136 - protein, 5 aa, synthetic construct
  REGION 1..5: note = C5-291 peptide selected for its ability to modulate theaggregation of the -amyloid peptide
TTLDR

SEQ ID NO: 137 - protein, 5 aa, synthetic construct
  REGION 1..5: note = C5-294 peptide selected for its ability to modulate theaggregation of the -amyloid peptide
TTPHR

SEQ ID NO: 138 - protein, 5 aa, synthetic construct
  REGION 1..5: note = C5-298 peptide selected for its ability to modulate theaggregation of the -amyloid peptide
TTRGR

SEQ ID NO: 139 - protein, 5 aa, synthetic construct
  REGION 1..5: note = C5-299 peptide selected for its ability to modulate theaggregation of the -amyloid peptide
TTVGR

SEQ ID NO: 140 - protein, 5 aa, synthetic construct
  REGION 1..5: note = C5-301 peptide selected for its ability to modulate theaggregation of the -amyloid peptide
TTTRR

SEQ ID NO: 141 - protein, 5 aa, synthetic construct
  REGION 1..5: note = C5-304 peptide selected for its ability to modulate theaggregation of the -amyloid peptide
TSINR

SEQ ID NO: 142 - protein, 5 aa, synthetic construct
  REGION 1..5: note = C5-305 peptide selected for its ability to modulate theaggregation of the -amyloid peptide
TTADR

SEQ ID NO: 143 - protein, 5 aa, synthetic construct
  REGION 1..5: note = C5-315 peptide selected for its ability to modulate theaggregation of the -amyloid peptide
TTSER

SEQ ID NO: 144 - protein, 5 aa, synthetic construct
  REGION 1..5: note = C5-316 peptide selected for its ability to modulate theaggregation of the -amyloid peptide
TTCAR

SEQ ID NO: 145 - protein, 5 aa, synthetic construct
  REGION 1..5: note = C5-317 peptide selected for its ability to modulate theaggregation of the -amyloid peptide
TTAWR

SEQ ID NO: 146 - protein, 5 aa, synthetic construct
  REGION 1..5: note = C5-320 peptide selected for its ability to modulate theaggregation of the -amyloid peptide
TTVER

SEQ ID NO: 147 - protein, 5 aa, synthetic construct
  REGION 1..5: note = C5-321 peptide selected for its ability to modulate theaggregation of the -amyloid peptide
TTTFR

SEQ ID NO: 148 - protein, 5 aa, synthetic construct
  REGION 1..5: note = C5-323 peptide selected for its ability to modulate theaggregation of the -amyloid peptide
TAVDR

SEQ ID NO: 149 - protein, 5 aa, synthetic construct
  REGION 1..5: note = C5-325 peptide selected for its ability to modulate theaggregation of the -amyloid peptide
TVWIR

SEQ ID NO: 150 - protein, 5 aa, synthetic construct
  REGION 1..5: note = C5-329 peptide selected for its ability to modulate theaggregation of the -amyloid peptide
TTVRR

SEQ ID NO: 151 - protein, 5 aa, synthetic construct
  REGION 1..5: note = C5-333 peptide selected for its ability to modulate theaggregation of the -amyloid peptide
THVRR

SEQ ID NO: 152 - protein, 5 aa, synthetic construct
  REGION 1..5: note = C5-343 peptide selected for its ability to modulate theaggregation of the -amyloid peptide
TNLDR

SEQ ID NO: 153 - protein, 5 aa, synthetic construct
  REGION 1..5: note = C5-344 peptide selected for its ability to modulate theaggregation of the -amyloid peptide
TTPGR

SEQ ID NO: 154 - protein, 5 aa, synthetic construct
  REGION 1..5: note = C5-348 peptide selected for its ability to modulate theaggregation of the -amyloid peptide
TTLTR

SEQ ID NO: 155 - protein, 5 aa, synthetic construct
  REGION 1..5: note = C5-355 peptide selected for its ability to modulate theaggregation of the -amyloid peptide
TATVR

SEQ ID NO: 156 - protein, 5 aa, synthetic construct
  REGION 1..5: note = C5-359 peptide selected for its ability to modulate theaggregation of the -amyloid peptide
TAMWR

SEQ ID NO: 157 - protein, 5 aa, synthetic construct
  REGION 1..5: note = C5-361 peptide selected for its ability to modulate theaggregation of the -amyloid peptide
TTKWR

SEQ ID NO: 158 - protein, 5 aa, synthetic construct
  REGION 1..5: note = C5-362 peptide selected for its ability to modulate theaggregation of the -amyloid peptide
TTWDR

SEQ ID NO: 159 - protein, 5 aa, synthetic construct
  REGION 1..5: note = C5-364 peptide selected for its ability to modulate theaggregation of the -amyloid peptide
TTMAR

SEQ ID NO: 160 - protein, 5 aa, synthetic construct
  REGION 1..5: note = C5-365 peptide selected for its ability to modulate theaggregation of the -amyloid peptide
TTGGR

SEQ ID NO: 161 - protein, 5 aa, synthetic construct
  REGION 1..5: note = C5-366 peptide selected for its ability to modulate theaggregation of the -amyloid peptide
TTMVR

SEQ ID NO: 162 - protein, 5 aa, synthetic construct
  REGION 1..5: note = C5-375 peptide selected for its ability to modulate theaggregation of the -amyloid peptide
TNLAR

SEQ ID NO: 163 - protein, 5 aa, synthetic construct
  REGION 1..5: note = C5-376 peptide selected for its ability to modulate theaggregation of the -amyloid peptide
TIRDR

SEQ ID NO: 164 - protein, 5 aa, synthetic construct
  REGION 1..5: note = C5-378 peptide selected for its ability to modulate theaggregation of the -amyloid peptide
TTTGR

SEQ ID NO: 165 - protein, 5 aa, synthetic construct
  REGION 1..5: note = C5-379 peptide selected for its ability to modulate theaggregation of the -amyloid peptide
TRLGR

SEQ ID NO: 166 - protein, 5 aa, synthetic construct
  REGION 1..5: note = C5-381 peptide selected for its ability to modulate theaggregation of the -amyloid peptide
TTHTR

SEQ ID NO: 167 - protein, 5 aa, synthetic construct
  REGION 1..5: note = C5-382 peptide selected for its ability to modulate theaggregation of the -amyloid peptide
TTITR

SEQ ID NO: 168 - protein, 5 aa, synthetic construct
  REGION 1..5: note = C5-384 peptide selected for its ability to modulate theaggregation of the -amyloid peptide
TTYTR

SEQ ID NO: 169 - protein, 5 aa, synthetic construct
  REGION 1..5: note = C5-385 peptide selected for its ability to modulate theaggregation of the -amyloid peptide
TTLYR

SEQ ID NO: 170 - protein, 5 aa, synthetic construct
  REGION 1..5: note = C5-389 peptide selected for its ability to modulate theaggregation of the -amyloid peptide
THLDR

SEQ ID NO: 171 - protein, 5 aa, synthetic construct
  REGION 1..5: note = C5-391 peptide selected for its ability to modulate theaggregation of the -amyloid peptide
TLLIR

SEQ ID NO: 172 - protein, 5 aa, synthetic construct
  REGION 1..5: note = C5-392 peptide selected for its ability to modulate theaggregation of the -amyloid peptide
TTCDR

SEQ ID NO: 173 - protein, 5 aa, synthetic construct
  REGION 1..5: note = C5-393 peptide selected for its ability to modulate theaggregation of the -amyloid peptide
TTGRR

SEQ ID NO: 174 - protein, 5 aa, synthetic construct
  REGION 1..5: note = C5-394 peptide selected for its ability to modulate theaggregation of the -amyloid peptide
TTVSR

SEQ ID NO: 175 - protein, 5 aa, synthetic construct
  REGION 1..5: note = C5-395 peptide selected for its ability to modulate theaggregation of the -amyloid peptide
TTQHR

SEQ ID NO: 176 - protein, 5 aa, synthetic construct
  REGION 1..5: note = C5-396 peptide selected for its ability to modulate theaggregation of the -amyloid peptide
TTTPR

SEQ ID NO: 177 - protein, 5 aa, synthetic construct
  REGION 1..5: note = C5-399 peptide selected for its ability to modulate theaggregation of the -amyloid peptide
TAFAR

SEQ ID NO: 178 - protein, 5 aa, synthetic construct
  REGION 1..5: note = C5-405 peptide selected for its ability to modulate theaggregation of the -amyloid peptide
TTSHR

SEQ ID NO: 179 - protein, 5 aa, synthetic construct
  REGION 1..5: note = C5-410 peptide selected for its ability to modulate theaggregation of the -amyloid peptide
TVLGR

SEQ ID NO: 180 - protein, 5 aa, synthetic construct
  REGION 1..5: note = C5-411 peptide selected for its ability to modulate theaggregation of the -amyloid peptide
TTQRR

SEQ ID NO: 181 - protein, 5 aa, synthetic construct
  REGION 1..5: note = C5-413 peptide selected for its ability to modulate theaggregation of the -amyloid peptide
TSHAR

SEQ ID NO: 182 - protein, 5 aa, synthetic construct
  REGION 1..5: note = C5-415 peptide selected for its ability to modulate theaggregation of the -amyloid peptide
TTTCR

SEQ ID NO: 183 - protein, 5 aa, synthetic construct
  REGION 1..5: note = C5-422 peptide selected for its ability to modulate theaggregation of the -amyloid peptide
TAWRR

SEQ ID NO: 184 - protein, 5 aa, synthetic construct
  REGION 1..5: note = C5-428 peptide selected for its ability to modulate theaggregation of the -amyloid peptide
TTCGR

SEQ ID NO: 185 - protein, 5 aa, synthetic construct
  REGION 1..5: note = C5-434 peptide selected for its ability to modulate theaggregation of the -amyloid peptide
TTSGR

SEQ ID NO: 186 - protein, 5 aa, synthetic construct
  REGION 1..5: note = C5-438 peptide selected for its ability to modulate theaggregation of the -amyloid peptide
TTTSR

SEQ ID NO: 187 - protein, 5 aa, synthetic construct
  REGION 1..5: note = C5-440 peptide selected for its ability to modulate theaggregation of the -amyloid peptide
TATGR

SEQ ID NO: 188 - protein, 5 aa, synthetic construct
  REGION 1..5: note = C5-441 peptide selected for its ability to modulate theaggregation of the -amyloid peptide
TAWDR

SEQ ID NO: 189 - protein, 5 aa, synthetic construct
  REGION 1..5: note = C5-443 peptide selected for its ability to modulate theaggregation of the -amyloid peptide
TTHHR

SEQ ID NO: 190 - protein, 5 aa, synthetic construct
  REGION 1..5: note = C5-448 peptide selected for its ability to modulate theaggregation of the -amyloid peptide
TAYAR

SEQ ID NO: 191 - protein, 5 aa, synthetic construct
  REGION 1..5: note = C5-449 peptide selected for its ability to modulate theaggregation of the -amyloid peptide
TANAR

SEQ ID NO: 192 - protein, 5 aa, synthetic construct
  REGION 1..5: note = C5-450 peptide selected for its ability to modulate theaggregation of the -amyloid peptide
TRDVR

SEQ ID NO: 193 - protein, 5 aa, synthetic construct
  REGION 1..5: note = C5-452 peptide selected for its ability to modulate theaggregation of the -amyloid peptide
THVDR

SEQ ID NO: 194 - protein, 5 aa, synthetic construct
  REGION 1..5: note = C5-453 peptide selected for its ability to modulate theaggregation of the -amyloid peptide
TLFWR

SEQ ID NO: 195 - protein, 5 aa, synthetic construct
  REGION 1..5: note = C5-459 peptide selected for its ability to modulate theaggregation of the -amyloid peptide
TTAAR

SEQ ID NO: 196 - protein, 5 aa, synthetic construct
  REGION 1..5: note = C5-463 peptide selected for its ability to modulate theaggregation of the -amyloid peptide
TVVDR

SEQ ID NO: 197 - protein, 5 aa, synthetic construct
  REGION 1..5: note = C5-464 peptide selected for its ability to modulate theaggregation of the -amyloid peptide
TTPAR

SEQ ID NO: 198 - protein, 5 aa, synthetic construct
  REGION 1..5: note = C5-469 peptide selected for its ability to modulate theaggregation of the -amyloid peptide
TTIGR

SEQ ID NO: 199 - protein, 5 aa, synthetic construct
  REGION 1..5: note = C5-472 peptide selected for its ability to modulate theaggregation of the -amyloid peptide
TMYAR

SEQ ID NO: 200 - protein, 5 aa, synthetic construct
  REGION 1..5: note = C5-473 peptide selected for its ability to modulate theaggregation of the -amyloid peptide
THVAR

SEQ ID NO: 201 - protein, 5 aa, synthetic construct
  REGION 1..5: note = C5-474 peptide selected for its ability to modulate theaggregation of the -amyloid peptide
TTWPR

SEQ ID NO: 202 - protein, 5 aa, synthetic construct
  REGION 1..5: note = C5-475 peptide selected for its ability to modulate theaggregation of the -amyloid peptide
TTGDR

SEQ ID NO: 203 - protein, 5 aa, synthetic construct
  REGION 1..5: note = C5-479 peptide selected for its ability to modulate theaggregation of the -amyloid peptide
TTTVR

SEQ ID NO: 204 - protein, 5 aa, synthetic construct
  REGION 1..5: note = C5-481 peptide selected for its ability to modulate theaggregation of the -amyloid peptide
TVFGR

SEQ ID NO: 205 - protein, 5 aa, synthetic construct
  REGION 1..5: note = C5-483 peptide selected for its ability to modulate theaggregation of the -amyloid peptide
TRVGR

SEQ ID NO: 206 - protein, 5 aa, synthetic construct
  REGION 1..5: note = C5-34 peptide selected for its ability to modulate theaggregation of the -amyloid peptide
SASPT

SEQ ID NO: 207 - protein, 5 aa, synthetic construct
  REGION 1..5: note = C5-216 peptide selected for its ability to modulate theaggregation of the -amyloid peptide
SICPT

SEQ ID NO: 208 - protein, 5 aa, synthetic construct
  REGION 1..5: note = C5-380 peptide selected for its ability to modulate theaggregation of the -amyloid peptide
SITPT

SEQ ID NO: 209 - protein, 5 aa, synthetic construct
  REGION 1..5: note = C5-387 peptide selected for its ability to modulate theaggregation of the -amyloid peptide
SHSPT

SEQ ID NO: 210 - protein, 4 aa, synthetic construct
  REGION 1..4: note = C4-9 peptide selected for its ability to modulate theaggregation of the -amyloid peptide
TTCR

SEQ ID NO: 211 - protein, 4 aa, synthetic construct
  REGION 1..4: note = C4-11 peptide selected for its ability to modulate theaggregation of the -amyloid peptide
TTRR

SEQ ID NO: 212 - protein, 4 aa, synthetic construct
  REGION 1..4: note = C4-31 peptide selected for its ability to modulate theaggregation of the -amyloid peptide
TTSR

SEQ ID NO: 213 - protein, 4 aa, synthetic construct
  REGION 1..4: note = C4-34 peptide selected for its ability to modulate theaggregation of the -amyloid peptide
TRGR

SEQ ID NO: 214 - protein, 4 aa, synthetic construct
  REGION 1..4: note = C4-35 peptide selected for its ability to modulate theaggregation of the -amyloid peptide
TTGR

SEQ ID NO: 215 - protein, 4 aa, synthetic construct
  REGION 1..4: note = C4-41 peptide selected for its ability to modulate theaggregation of the -amyloid peptide
TRRR

SEQ ID NO: 216 - protein, 4 aa, synthetic construct
  REGION 1..4: note = AC4B-9 peptide selected for its ability to modulate theaggregation of the -amyloid peptide
TDQR

SEQ ID NO: 217 - protein, 4 aa, synthetic construct
  REGION 1..4: note = AC4B-41 peptide selected for its ability to modulate theaggregation of the -amyloid peptide
TLIR

SEQ ID NO: 218 - protein, 4 aa, synthetic construct
  REGION 1..4: note = AC4B-80 peptide selected for its ability to modulate theaggregation of the -amyloid peptide
TLWR

SEQ ID NO: 219 - protein, 4 aa, synthetic construct
  REGION 1..4: note = AC4B-86 peptide selected for its ability to modulate theaggregation of the -amyloid peptide
TLGR

SEQ ID NO: 220 - protein, 4 aa, synthetic construct
  REGION 1..4: note = C5(2) peptide selected for its ability to modulate theaggregation of the -amyloid peptide
TFDR

SEQ ID NO: 221 - protein, 4 aa, synthetic construct
  REGION 1..4: note = C5(D4) peptide selected for its ability to modulate theaggregation of the -amyloid peptide
TAFR

SEQ ID NO: 222 - protein, 6 aa, synthetic construct
  REGION 1..6: note = AC6-1 peptide selected for its ability to modulate theaggregation of the -amyloid peptide
TPVWFD

SEQ ID NO: 223 - protein, 6 aa, synthetic construct
  REGION 1..6: note = AC6-2 peptide selected for its ability to modulate theaggregation of the -amyloid peptide
TPAWFD

SEQ ID NO: 224 - protein, 6 aa, synthetic construct
  REGION 1..6: note = AC6-4 peptide selected for its ability to modulate theaggregation of the -amyloid peptide
TLEFFD

SEQ ID NO: 225 - protein, 6 aa, synthetic construct
  REGION 1..6: note = AC6-6 peptide selected for its ability to modulate theaggregation of the -amyloid peptide
TVTWFD

SEQ ID NO: 226 - protein, 6 aa, synthetic construct
  REGION 1..6: note = AC6-8 peptide selected for its ability to modulate theaggregation of the -amyloid peptide
TLLIRW

SEQ ID NO: 227 - protein, 6 aa, synthetic construct
  REGION 1..6: note = AC6-10 peptide selected for its ability to modulate theaggregation of the -amyloid peptide
TLKWLN

SEQ ID NO: 228 - protein, 6 aa, synthetic construct
  REGION 1..6: note = AC6-21 peptide selected for its ability to modulate theaggregation of the -amyloid peptide
TKEYFD

SEQ ID NO: 229 - protein, 6 aa, synthetic construct
  REGION 1..6: note = AC6-26 peptide selected for its ability to modulate theaggregation of the -amyloid peptide
TLHWFE

SEQ ID NO: 230 - protein, 6 aa, synthetic construct
  REGION 1..6: note = AC6-27 peptide selected for its ability to modulate theaggregation of the -amyloid peptide
TCSWFD

SEQ ID NO: 231 - protein, 6 aa, synthetic construct
  REGION 1..6: note = AC6-28 peptide selected for its ability to modulate theaggregation of the -amyloid peptide
TLEYFM

SEQ ID NO: 232 - protein, 6 aa, synthetic construct
  REGION 1..6: note = AC6-32 peptide selected for its ability to modulate theaggregation of the -amyloid peptide
TLCWLN

SEQ ID NO: 233 - protein, 6 aa, synthetic construct
  REGION 1..6: note = AC6-36 peptide selected for its ability to modulate theaggregation of the -amyloid peptide
TPIVFD

SEQ ID NO: 234 - protein, 6 aa, synthetic construct
  REGION 1..6: note = AC6-37 peptide selected for its ability to modulate theaggregation of the -amyloid peptide
TLWVFD

SEQ ID NO: 235 - protein, 6 aa, synthetic construct
  REGION 1..6: note = AC6-40 peptide selected for its ability to modulate theaggregation of the -amyloid peptide
TPLWFN

SEQ ID NO: 236 - protein, 6 aa, synthetic construct
  REGION 1..6: note = AC6-41 peptide selected for its ability to modulate theaggregation of the -amyloid peptide
TSVEYE

SEQ ID NO: 237 - protein, 6 aa, synthetic construct
  REGION 1..6: note = AC6-42 peptide selected for its ability to modulate theaggregation of the -amyloid peptide
TLGWLD

SEQ ID NO: 238 - protein, 6 aa, synthetic construct
  REGION 1..6: note = AC6-44 peptide selected for its ability to modulate theaggregation of the -amyloid peptide
TPPWFD

SEQ ID NO: 239 - protein, 6 aa, synthetic construct
  REGION 1..6: note = AC6-46 peptide selected for its ability to modulate theaggregation of the -amyloid peptide
TPCWFD

SEQ ID NO: 240 - protein, 6 aa, synthetic construct
  REGION 1..6: note = AC6-47 peptide selected for its ability to modulate theaggregation of the -amyloid peptide
TLSWYD

SEQ ID NO: 241 - protein, 6 aa, synthetic construct
  REGION 1..6: note = AC6-48 peptide selected for its ability to modulate theaggregation of the -amyloid peptide
TPVLVD

SEQ ID NO: 242 - protein, 6 aa, synthetic construct
  REGION 1..6: note = AC6-49 peptide selected for its ability to modulate theaggregation of the -amyloid peptide
TLEYLW

SEQ ID NO: 243 - protein, 6 aa, synthetic construct
  REGION 1..6: note = AC6-50 peptide selected for its ability to modulate theaggregation of the -amyloid peptide
TIFWFD

SEQ ID NO: 244 - protein, 6 aa, synthetic construct
  REGION 1..6: note = AC6-53 peptide selected for its ability to modulate theaggregation of the -amyloid peptide
TPALVD

SEQ ID NO: 245 - protein, 6 aa, synthetic construct
  REGION 1..6: note = AC6-55 peptide selected for its ability to modulate theaggregation of the -amyloid peptide
TPGWFD

SEQ ID NO: 246 - protein, 6 aa, synthetic construct
  REGION 1..6: note = AC6-57 peptide selected for its ability to modulate theaggregation of the -amyloid peptide
TLSVFD

SEQ ID NO: 247 - protein, 6 aa, synthetic construct
  REGION 1..6: note = AC6-58 peptide selected for its ability to modulate theaggregation of the -amyloid peptide
TPGLVD

SEQ ID NO: 248 - protein, 6 aa, synthetic construct
  REGION 1..6: note = AC6-59 peptide selected for its ability to modulate theaggregation of the -amyloid peptide
TLSWFN

SEQ ID NO: 249 - protein, 6 aa, synthetic construct
  REGION 1..6: note = AC6-63 peptide selected for its ability to modulate theaggregation of the -amyloid peptide
TLDFFD

SEQ ID NO: 250 - protein, 6 aa, synthetic construct
  REGION 1..6: note = AC6-65 peptide selected for its ability to modulate theaggregation of the -amyloid peptide
TPSWFD

SEQ ID NO: 251 - protein, 6 aa, synthetic construct
  REGION 1..6: note = AC6-68 peptide selected for its ability to modulate theaggregation of the -amyloid peptide
TPALFD

SEQ ID NO: 252 - protein, 6 aa, synthetic construct
  REGION 1..6: note = AC6-69 peptide selected for its ability to modulate theaggregation of the -amyloid peptide
TPAWSD

SEQ ID NO: 253 - protein, 6 aa, synthetic construct
  REGION 1..6: note = AC6-78 peptide selected for its ability to modulate theaggregation of the -amyloid peptide
TPARFD

SEQ ID NO: 254 - protein, 6 aa, synthetic construct
  REGION 1..6: note = AC6-79 peptide selected for its ability to modulate theaggregation of the -amyloid peptide
TPAWLD

SEQ ID NO: 255 - protein, 6 aa, synthetic construct
  REGION 1..6: note = AC6-80 peptide selected for its ability to modulate theaggregation of the -amyloid peptide
TPVWLD

SEQ ID NO: 256 - DNA, 15 bp, synthetic construct
  misc_feature 1..15: note = >DNA sequence encoding for cyclic peptide C5-2
  source 1..15: mol_type = other DNA
accacgtacgccagg

SEQ ID NO: 257 - DNA, 15 bp, synthetic construct
  misc_feature 1..15: note = >DNA sequence encoding for cyclic peptide C5-3
  source 1..15: mol_type = other DNA
accaccgtggaccgg

SEQ ID NO: 258 - DNA, 15 bp, synthetic construct
  misc_feature 1..15: note = >DNA sequence encoding for cyclic peptide C5-5
  source 1..15: mol_type = other DNA
accacgacctggagg

SEQ ID NO: 259 - DNA, 15 bp, synthetic construct
  misc_feature 1..15: note = >DNA sequence encoding for cyclic peptide C5-7
  source 1..15: mol_type = other DNA
accacgctgcaccgg

SEQ ID NO: 260 - DNA, 15 bp, synthetic construct
  misc_feature 1..15: note = >DNA sequence encoding for cyclic peptide C5-8
  source 1..15: mol_type = other DNA
accaccttcgcccgg

SEQ ID NO: 261 - DNA, 15 bp, synthetic construct
  misc_feature 1..15: note = >DNA sequence encoding for cyclic peptide C5-9
  source 1..15: mol_type = other DNA
accgtcttggaccgg

SEQ ID NO: 262 - DNA, 15 bp, synthetic construct
  misc_feature 1..15: note = >DNA sequence encoding for cyclic peptide C5-12
  source 1..15: mol_type = other DNA
accacgtgggccagg

SEQ ID NO: 263 - DNA, 15 bp, synthetic construct
  misc_feature 1..15: note = >DNA sequence encoding for cyclic peptide C5-13
  source 1..15: mol_type = other DNA
accgcgctggaccgg

SEQ ID NO: 264 - DNA, 15 bp, synthetic construct
  misc_feature 1..15: note = >DNA sequence encoding for cyclic peptide C5-15
  source 1..15: mol_type = other DNA
accgcgaacgtgagg

SEQ ID NO: 265 - DNA, 15 bp, synthetic construct
  misc_feature 1..15: note = >DNA sequence encoding for cyclic peptide C5-17
  source 1..15: mol_type = other DNA
accaccacggcccgg

SEQ ID NO: 266 - DNA, 15 bp, synthetic construct
  misc_feature 1..15: note = >DNA sequence encoding for cyclic peptide C5-18
  source 1..15: mol_type = other DNA
accaccatcgcccgg

SEQ ID NO: 267 - DNA, 15 bp, synthetic construct
  misc_feature 1..15: note = >DNA sequence encoding for cyclic peptide C5-19
  source 1..15: mol_type = other DNA
accgtgtgggaccgg

SEQ ID NO: 268 - DNA, 15 bp, synthetic construct
  misc_feature 1..15: note = >DNA sequence encoding for cyclic peptide C5-20
  source 1..15: mol_type = other DNA
accaccatcagccgg

SEQ ID NO: 269 - DNA, 15 bp, synthetic construct
  misc_feature 1..15: note = >DNA sequence encoding for cyclic peptide C5-21
  source 1..15: mol_type = other DNA
accacctggtgccgg

SEQ ID NO: 270 - DNA, 15 bp, synthetic construct
  misc_feature 1..15: note = >DNA sequence encoding for cyclic peptide C5-22
  source 1..15: mol_type = other DNA
accgtcctgtggagg

SEQ ID NO: 271 - DNA, 15 bp, synthetic construct
  misc_feature 1..15: note = >DNA sequence encoding for cyclic peptide C5-25
  source 1..15: mol_type = other DNA
accaccttggcgagg

SEQ ID NO: 272 - DNA, 15 bp, synthetic construct
  misc_feature 1..15: note = >DNA sequence encoding for cyclic peptide C5-26
  source 1..15: mol_type = other DNA
accgcgtggtgccgc

SEQ ID NO: 273 - DNA, 15 bp, synthetic construct
  misc_feature 1..15: note = >DNA sequence encoding for cyclic peptide C5-27
  source 1..15: mol_type = other DNA
accacgagcgcccgc

SEQ ID NO: 274 - DNA, 15 bp, synthetic construct
  misc_feature 1..15: note = >DNA sequence encoding for cyclic peptide C5-29
  source 1..15: mol_type = other DNA
accaccctcgagagg

SEQ ID NO: 275 - DNA, 15 bp, synthetic construct
  misc_feature 1..15: note = >DNA sequence encoding for cyclic peptide C5-30
  source 1..15: mol_type = other DNA
acctcgacggcgcgg

SEQ ID NO: 276 - DNA, 15 bp, synthetic construct
  misc_feature 1..15: note = >DNA sequence encoding for cyclic peptide C5-34
  source 1..15: mol_type = other DNA
agcgcctcgccgacg

SEQ ID NO: 277 - DNA, 15 bp, synthetic construct
  misc_feature 1..15: note = >DNA sequence encoding for cyclic peptide C5-35
  source 1..15: mol_type = other DNA
accgtccgggaccgg

SEQ ID NO: 278 - DNA, 15 bp, synthetic construct
  misc_feature 1..15: note = >DNA sequence encoding for cyclic peptide C5-41
  source 1..15: mol_type = other DNA
accggctgggcgagg

SEQ ID NO: 279 - DNA, 15 bp, synthetic construct
  misc_feature 1..15: note = >DNA sequence encoding for cyclic peptide C5-44
  source 1..15: mol_type = other DNA
accgcctgggcgagg

SEQ ID NO: 280 - DNA, 15 bp, synthetic construct
  misc_feature 1..15: note = >DNA sequence encoding for cyclic peptide C5-45
  source 1..15: mol_type = other DNA
accacctgggtgcgg

SEQ ID NO: 281 - DNA, 15 bp, synthetic construct
  misc_feature 1..15: note = >DNA sequence encoding for cyclic peptide C5-46
  source 1..15: mol_type = other DNA
accctattgtggcgg

SEQ ID NO: 282 - DNA, 15 bp, synthetic construct
  misc_feature 1..15: note = >DNA sequence encoding for cyclic peptide C5-47
  source 1..15: mol_type = other DNA
accacgatcgacagg

SEQ ID NO: 283 - DNA, 15 bp, synthetic construct
  misc_feature 1..15: note = >DNA sequence encoding for cyclic peptide C5-50
  source 1..15: mol_type = other DNA
accgcgctcgcgcgc

SEQ ID NO: 284 - DNA, 15 bp, synthetic construct
  misc_feature 1..15: note = >DNA sequence encoding for cyclic peptide C5-51
  source 1..15: mol_type = other DNA
accagcgtggacagg

SEQ ID NO: 285 - DNA, 15 bp, synthetic construct
  misc_feature 1..15: note = >DNA sequence encoding for cyclic peptide C5-53
  source 1..15: mol_type = other DNA
accaccgtgtggcgc

SEQ ID NO: 286 - DNA, 15 bp, synthetic construct
  misc_feature 1..15: note = >DNA sequence encoding for cyclic peptide C5-66
  source 1..15: mol_type = other DNA
accacgcactggcgg

SEQ ID NO: 287 - DNA, 15 bp, synthetic construct
  misc_feature 1..15: note = >DNA sequence encoding for cyclic peptide C5-67
  source 1..15: mol_type = other DNA
accgcgagggaccgg

SEQ ID NO: 288 - DNA, 15 bp, synthetic construct
  misc_feature 1..15: note = >DNA sequence encoding for cyclic peptide C5-73
  source 1..15: mol_type = other DNA
accacgcgggaccgg

SEQ ID NO: 289 - DNA, 15 bp, synthetic construct
  misc_feature 1..15: note = >DNA sequence encoding for cyclic peptide C5-80
  source 1..15: mol_type = other DNA
accagcgtgcaccgg

SEQ ID NO: 290 - DNA, 15 bp, synthetic construct
  misc_feature 1..15: note = >DNA sequence encoding for cyclic peptide C5-82
  source 1..15: mol_type = other DNA
accgccgtctggcgg

SEQ ID NO: 291 - DNA, 15 bp, synthetic construct
  misc_feature 1..15: note = >DNA sequence encoding for cyclic peptide C5-83
  source 1..15: mol_type = other DNA
accacggggtgccgg

SEQ ID NO: 292 - DNA, 15 bp, synthetic construct
  misc_feature 1..15: note = >DNA sequence encoding for cyclic peptide C5-89
  source 1..15: mol_type = other DNA
accgccaccgacagg

SEQ ID NO: 293 - DNA, 15 bp, synthetic construct
  misc_feature 1..15: note = >DNA sequence encoding for cyclic peptide C5-94
  source 1..15: mol_type = other DNA
accgtcttgttccgc

SEQ ID NO: 294 - DNA, 15 bp, synthetic construct
  misc_feature 1..15: note = >DNA sequence encoding for cyclic peptide C5-102
  source 1..15: mol_type = other DNA
accacctacaaccgc

SEQ ID NO: 295 - DNA, 15 bp, synthetic construct
  misc_feature 1..15: note = >DNA sequence encoding for cyclic peptide C5-105
  source 1..15: mol_type = other DNA
accgtgcgctggcgc

SEQ ID NO: 296 - DNA, 15 bp, synthetic construct
  misc_feature 1..15: note = >DNA sequence encoding for cyclic peptide C5-116
  source 1..15: mol_type = other DNA
accgcgttcgaccgg

SEQ ID NO: 297 - DNA, 15 bp, synthetic construct
  misc_feature 1..15: note = >DNA sequence encoding for cyclic peptide C5-117
  source 1..15: mol_type = other DNA
accacgcggtgcagg

SEQ ID NO: 298 - DNA, 15 bp, synthetic construct
  misc_feature 1..15: note = >DNA sequence encoding for cyclic peptide C5-118
  source 1..15: mol_type = other DNA
accaccttctggcgg

SEQ ID NO: 299 - DNA, 15 bp, synthetic construct
  misc_feature 1..15: note = >DNA sequence encoding for cyclic peptide C5-121
  source 1..15: mol_type = other DNA
accatcaaggaccgg

SEQ ID NO: 300 - DNA, 15 bp, synthetic construct
  misc_feature 1..15: note = >DNA sequence encoding for cyclic peptide C5-123
  source 1..15: mol_type = other DNA
accaccgtccaccgg

SEQ ID NO: 301 - DNA, 15 bp, synthetic construct
  misc_feature 1..15: note = >DNA sequence encoding for cyclic peptide C5-126
  source 1..15: mol_type = other DNA
accacgctcctcagg

SEQ ID NO: 302 - DNA, 15 bp, synthetic construct
  misc_feature 1..15: note = >DNA sequence encoding for cyclic peptide C5-129
  source 1..15: mol_type = other DNA
accacgctcttccgg

SEQ ID NO: 303 - DNA, 15 bp, synthetic construct
  misc_feature 1..15: note = >DNA sequence encoding for cyclic peptide C5-130
  source 1..15: mol_type = other DNA
accgcgtaccaccgg

SEQ ID NO: 304 - DNA, 15 bp, synthetic construct
  misc_feature 1..15: note = >DNA sequence encoding for cyclic peptide C5-136
  source 1..15: mol_type = other DNA
accgcgttgcaccgg

SEQ ID NO: 305 - DNA, 15 bp, synthetic construct
  misc_feature 1..15: note = >DNA sequence encoding for cyclic peptide C5-139
  source 1..15: mol_type = other DNA
accacctcgccccgg

SEQ ID NO: 306 - DNA, 15 bp, synthetic construct
  misc_feature 1..15: note = >DNA sequence encoding for cyclic peptide C5-146
  source 1..15: mol_type = other DNA
accacctggtcgcgg

SEQ ID NO: 307 - DNA, 15 bp, synthetic construct
  misc_feature 1..15: note = >DNA sequence encoding for cyclic peptide C5-147
  source 1..15: mol_type = other DNA
accgccatgcacagg

SEQ ID NO: 308 - DNA, 15 bp, synthetic construct
  misc_feature 1..15: note = >DNA sequence encoding for cyclic peptide C5-155
  source 1..15: mol_type = other DNA
acctcgctcgacagg

SEQ ID NO: 309 - DNA, 15 bp, synthetic construct
  misc_feature 1..15: note = >DNA sequence encoding for cyclic peptide C5-158
  source 1..15: mol_type = other DNA
accacgggggcgcgc

SEQ ID NO: 310 - DNA, 15 bp, synthetic construct
  misc_feature 1..15: note = >DNA sequence encoding for cyclic peptide C5-162
  source 1..15: mol_type = other DNA
acctcggtgtggagg

SEQ ID NO: 311 - DNA, 15 bp, synthetic construct
  misc_feature 1..15: note = >DNA sequence encoding for cyclic peptide C5-173
  source 1..15: mol_type = other DNA
accacgcacgccagg

SEQ ID NO: 312 - DNA, 15 bp, synthetic construct
  misc_feature 1..15: note = >DNA sequence encoding for cyclic peptide C5-176
  source 1..15: mol_type = other DNA
accgcgggctggagg

SEQ ID NO: 313 - DNA, 15 bp, synthetic construct
  misc_feature 1..15: note = >DNA sequence encoding for cyclic peptide C5-177
  source 1..15: mol_type = other DNA
accgccaccgcgagg

SEQ ID NO: 314 - DNA, 15 bp, synthetic construct
  misc_feature 1..15: note = >DNA sequence encoding for cyclic peptide C5-184
  source 1..15: mol_type = other DNA
accgtgctcgcgcgg

SEQ ID NO: 315 - DNA, 15 bp, synthetic construct
  misc_feature 1..15: note = >DNA sequence encoding for cyclic peptide C5-185
  source 1..15: mol_type = other DNA
accacgttcaacagg

SEQ ID NO: 316 - DNA, 15 bp, synthetic construct
  misc_feature 1..15: note = >DNA sequence encoding for cyclic peptide C5-188
  source 1..15: mol_type = other DNA
accgggatgaggcgg

SEQ ID NO: 317 - DNA, 15 bp, synthetic construct
  misc_feature 1..15: note = >DNA sequence encoding for cyclic peptide C5-189
  source 1..15: mol_type = other DNA
accaccgtcgccagg

SEQ ID NO: 318 - DNA, 15 bp, synthetic construct
  misc_feature 1..15: note = >DNA sequence encoding for cyclic peptide A C5-190
  source 1..15: mol_type = other DNA
tgcttgcgcacgctg

SEQ ID NO: 319 - DNA, 15 bp, synthetic construct
  misc_feature 1..15: note = >DNA sequence encoding for cyclic peptide C5-192
  source 1..15: mol_type = other DNA
accgggctggcgcgg

SEQ ID NO: 320 - DNA, 15 bp, synthetic construct
  misc_feature 1..15: note = >DNA sequence encoding for cyclic peptide C5-198
  source 1..15: mol_type = other DNA
accagctggtgcagg

SEQ ID NO: 321 - DNA, 15 bp, synthetic construct
  misc_feature 1..15: note = >DNA sequence encoding for cyclic peptide C5-209
  source 1..15: mol_type = other DNA
accaccagggcgcgg

SEQ ID NO: 322 - DNA, 15 bp, synthetic construct
  misc_feature 1..15: note = >DNA sequence encoding for cyclic peptide C5-215
  source 1..15: mol_type = other DNA
accacgccctggagg

SEQ ID NO: 323 - DNA, 15 bp, synthetic construct
  misc_feature 1..15: note = >DNA sequence encoding for cyclic peptide C5-218
  source 1..15: mol_type = other DNA
accgtcttgcacagg

SEQ ID NO: 324 - DNA, 15 bp, synthetic construct
  misc_feature 1..15: note = >DNA sequence encoding for cyclic peptide C5-223
  source 1..15: mol_type = other DNA
accggcctcgacagg

SEQ ID NO: 325 - DNA, 15 bp, synthetic construct
  misc_feature 1..15: note = >DNA sequence encoding for cyclic peptide C5-230
  source 1..15: mol_type = other DNA
accacgtcggaccgg

SEQ ID NO: 326 - DNA, 15 bp, synthetic construct
  misc_feature 1..15: note = >DNA sequence encoding for cyclic peptide C5-239
  source 1..15: mol_type = other DNA
accacgatgcaccgc

SEQ ID NO: 327 - DNA, 15 bp, synthetic construct
  misc_feature 1..15: note = >DNA sequence encoding for cyclic peptide C5-242
  source 1..15: mol_type = other DNA
accacctcgacccgg

SEQ ID NO: 328 - DNA, 15 bp, synthetic construct
  misc_feature 1..15: note = >DNA sequence encoding for cyclic peptide C5-244
  source 1..15: mol_type = other DNA
accacgcgcgtgagg

SEQ ID NO: 329 - DNA, 15 bp, synthetic construct
  misc_feature 1..15: note = >DNA sequence encoding for cyclic peptide C5-245
  source 1..15: mol_type = other DNA
accacccggttccgg

SEQ ID NO: 330 - DNA, 15 bp, synthetic construct
  misc_feature 1..15: note = >DNA sequence encoding for cyclic peptide C5-248
  source 1..15: mol_type = other DNA
accacgacgcaccgg

SEQ ID NO: 331 - DNA, 15 bp, synthetic construct
  misc_feature 1..15: note = >DNA sequence encoding for cyclic peptide C5-250
  source 1..15: mol_type = other DNA
acccacgcctggagg

SEQ ID NO: 332 - DNA, 15 bp, synthetic construct
  misc_feature 1..15: note = >DNA sequence encoding for cyclic peptide C5-252
  source 1..15: mol_type = other DNA
accgtgatctggcgc

SEQ ID NO: 333 - DNA, 15 bp, synthetic construct
  misc_feature 1..15: note = >DNA sequence encoding for cyclic peptide C5-253
  source 1..15: mol_type = other DNA
accacgtggttccgg

SEQ ID NO: 334 - DNA, 15 bp, synthetic construct
  misc_feature 1..15: note = >DNA sequence encoding for cyclic peptide C5-255
  source 1..15: mol_type = other DNA
accacctcgagacgg

SEQ ID NO: 335 - DNA, 15 bp, synthetic construct
  misc_feature 1..15: note = >DNA sequence encoding for cyclic peptide C5-258
  source 1..15: mol_type = other DNA
accacgtcgtgccgg

SEQ ID NO: 336 - DNA, 15 bp, synthetic construct
  misc_feature 1..15: note = >DNA sequence encoding for cyclic peptide C5-260
  source 1..15: mol_type = other DNA
accacctggacccgg

SEQ ID NO: 337 - DNA, 15 bp, synthetic construct
  misc_feature 1..15: note = >DNA sequence encoding for cyclic peptide C5-262
  source 1..15: mol_type = other DNA
accacctcgagccgg

SEQ ID NO: 338 - DNA, 15 bp, synthetic construct
  misc_feature 1..15: note = >DNA sequence encoding for cyclic peptide C5-263
  source 1..15: mol_type = other DNA
acccacctcgcccgg

SEQ ID NO: 339 - DNA, 15 bp, synthetic construct
  misc_feature 1..15: note = >DNA sequence encoding for cyclic peptide C5-264
  source 1..15: mol_type = other DNA
accagcggggcccgg

SEQ ID NO: 340 - DNA, 15 bp, synthetic construct
  misc_feature 1..15: note = >DNA sequence encoding for cyclic peptide C5-266
  source 1..15: mol_type = other DNA
accacgctgcgccgg

SEQ ID NO: 341 - DNA, 15 bp, synthetic construct
  misc_feature 1..15: note = >DNA sequence encoding for cyclic peptide C5-270
  source 1..15: mol_type = other DNA
accgcgacctggagg

SEQ ID NO: 342 - DNA, 15 bp, synthetic construct
  misc_feature 1..15: note = >DNA sequence encoding for cyclic peptide C5-272
  source 1..15: mol_type = other DNA
acctgcatgtggcgc

SEQ ID NO: 343 - DNA, 15 bp, synthetic construct
  misc_feature 1..15: note = >DNA sequence encoding for cyclic peptide C5-275
  source 1..15: mol_type = other DNA
accgcgcacgtgcgc

SEQ ID NO: 344 - DNA, 15 bp, synthetic construct
  misc_feature 1..15: note = >DNA sequence encoding for cyclic peptide C5-276
  source 1..15: mol_type = other DNA
acctcgtgggcgcgg

SEQ ID NO: 345 - DNA, 15 bp, synthetic construct
  misc_feature 1..15: note = >DNA sequence encoding for cyclic peptide C5-278
  source 1..15: mol_type = other DNA
accacgtggctcagg

SEQ ID NO: 346 - DNA, 15 bp, synthetic construct
  misc_feature 1..15: note = >DNA sequence encoding for cyclic peptide C5-291
  source 1..15: mol_type = other DNA
accaccctggaccgg

SEQ ID NO: 347 - DNA, 15 bp, synthetic construct
  misc_feature 1..15: note = >DNA sequence encoding for cyclic peptide C5-294
  source 1..15: mol_type = other DNA
accacgcctcaccgg

SEQ ID NO: 348 - DNA, 15 bp, synthetic construct
  misc_feature 1..15: note = >DNA sequence encoding for cyclic peptide C5-298
  source 1..15: mol_type = other DNA
accacccgtggccgg

SEQ ID NO: 349 - DNA, 15 bp, synthetic construct
  misc_feature 1..15: note = >DNA sequence encoding for cyclic peptide C5-299
  source 1..15: mol_type = other DNA
accaccgtgggccgg

SEQ ID NO: 350 - DNA, 15 bp, synthetic construct
  misc_feature 1..15: note = >DNA sequence encoding for cyclic peptide C5-301
  source 1..15: mol_type = other DNA
accacgacgcgccgc

SEQ ID NO: 351 - DNA, 15 bp, synthetic construct
  misc_feature 1..15: note = >DNA sequence encoding for cyclic peptide C5-304
  source 1..15: mol_type = other DNA
acctcgatcaacagg

SEQ ID NO: 352 - DNA, 15 bp, synthetic construct
  misc_feature 1..15: note = >DNA sequence encoding for cyclic peptide C5-305
  source 1..15: mol_type = other DNA
accaccgcggaccgg

SEQ ID NO: 353 - DNA, 15 bp, synthetic construct
  misc_feature 1..15: note = >DNA sequence encoding for cyclic peptide C5-315
  source 1..15: mol_type = other DNA
accacctccgagagg

SEQ ID NO: 354 - DNA, 15 bp, synthetic construct
  misc_feature 1..15: note = >DNA sequence encoding for cyclic peptide C5-316
  source 1..15: mol_type = other DNA
accacgtgcgccagg

SEQ ID NO: 355 - DNA, 15 bp, synthetic construct
  misc_feature 1..15: note = >DNA sequence encoding for cyclic peptide C5-317
  source 1..15: mol_type = other DNA
accacggcctggagg

SEQ ID NO: 356 - DNA, 15 bp, synthetic construct
  misc_feature 1..15: note = >DNA sequence encoding for cyclic peptide C5-320
  source 1..15: mol_type = other DNA
accaccgtcgagcgg

SEQ ID NO: 357 - DNA, 15 bp, synthetic construct
  misc_feature 1..15: note = >DNA sequence encoding for cyclic peptide C5-321
  source 1..15: mol_type = other DNA
accacgacgttcagg

SEQ ID NO: 358 - DNA, 15 bp, synthetic construct
  misc_feature 1..15: note = >DNA sequence encoding for cyclic peptide C5-323
  source 1..15: mol_type = other DNA
accgccgtggaccgg

SEQ ID NO: 359 - DNA, 15 bp, synthetic construct
  misc_feature 1..15: note = >DNA sequence encoding for cyclic peptide C5-325
  source 1..15: mol_type = other DNA
accgtgtggatcagg

SEQ ID NO: 360 - DNA, 15 bp, synthetic construct
  misc_feature 1..15: note = >DNA sequence encoding for cyclic peptide C5-329
  source 1..15: mol_type = other DNA
accaccgtacgcagg

SEQ ID NO: 361 - DNA, 15 bp, synthetic construct
  misc_feature 1..15: note = >DNA sequence encoding for cyclic peptide C5-333
  source 1..15: mol_type = other DNA
acccacgtacgcagg

SEQ ID NO: 362 - DNA, 15 bp, synthetic construct
  misc_feature 1..15: note = >DNA sequence encoding for cyclic peptide C5-343
  source 1..15: mol_type = other DNA
accaacctggaccgg

SEQ ID NO: 363 - DNA, 15 bp, synthetic construct
  misc_feature 1..15: note = >DNA sequence encoding for cyclic peptide C5-344
  source 1..15: mol_type = other DNA
accacgcctggacgg

SEQ ID NO: 364 - DNA, 15 bp, synthetic construct
  misc_feature 1..15: note = >DNA sequence encoding for cyclic peptide C5-348
  source 1..15: mol_type = other DNA
accacgctcacccgg

SEQ ID NO: 365 - DNA, 15 bp, synthetic construct
  misc_feature 1..15: note = >DNA sequence encoding for cyclic peptide C5-355
  source 1..15: mol_type = other DNA
accgcgacggtgcgc

SEQ ID NO: 366 - DNA, 15 bp, synthetic construct
  misc_feature 1..15: note = >DNA sequence encoding for cyclic peptide C5-359
  source 1..15: mol_type = other DNA
accgccatgtggcgg

SEQ ID NO: 367 - DNA, 15 bp, synthetic construct
  misc_feature 1..15: note = >DNA sequence encoding for cyclic peptide C5-361
  source 1..15: mol_type = other DNA
accacgaagtggagg

SEQ ID NO: 368 - DNA, 15 bp, synthetic construct
  misc_feature 1..15: note = >DNA sequence encoding for cyclic peptide C5-362
  source 1..15: mol_type = other DNA
accacctgggaccgg

SEQ ID NO: 369 - DNA, 15 bp, synthetic construct
  misc_feature 1..15: note = >DNA sequence encoding for cyclic peptide C5-364
  source 1..15: mol_type = other DNA
accaccatggcccgg

SEQ ID NO: 370 - DNA, 15 bp, synthetic construct
  misc_feature 1..15: note = >DNA sequence encoding for cyclic peptide C5-365
  source 1..15: mol_type = other DNA
accaccggtggccgg

SEQ ID NO: 371 - DNA, 15 bp, synthetic construct
  misc_feature 1..15: note = >DNA sequence encoding for cyclic peptide C5-366
  source 1..15: mol_type = other DNA
accacgatggtgcgg

SEQ ID NO: 372 - DNA, 15 bp, synthetic construct
  misc_feature 1..15: note = >DNA sequence encoding for cyclic peptide C5-375
  source 1..15: mol_type = other DNA
accaacctcgcccgg

SEQ ID NO: 373 - DNA, 15 bp, synthetic construct
  misc_feature 1..15: note = >DNA sequence encoding for cyclic peptide C5-376
  source 1..15: mol_type = other DNA
accatcagggaccgg

SEQ ID NO: 374 - DNA, 15 bp, synthetic construct
  misc_feature 1..15: note = >DNA sequence encoding for cyclic peptide C5-378
  source 1..15: mol_type = other DNA
accacgactggtagg

SEQ ID NO: 375 - DNA, 15 bp, synthetic construct
  misc_feature 1..15: note = >DNA sequence encoding for cyclic peptide C5-379
  source 1..15: mol_type = other DNA
acccgtcttggcagg

SEQ ID NO: 376 - DNA, 15 bp, synthetic construct
  misc_feature 1..15: note = >DNA sequence encoding for cyclic peptide C5-381
  source 1..15: mol_type = other DNA
accacgcacaccagg

SEQ ID NO: 377 - DNA, 15 bp, synthetic construct
  misc_feature 1..15: note = >DNA sequence encoding for cyclic peptide C5-382
  source 1..15: mol_type = other DNA
accaccatcacccgg

SEQ ID NO: 378 - DNA, 15 bp, synthetic construct
  misc_feature 1..15: note = >DNA sequence encoding for cyclic peptide C5-384
  source 1..15: mol_type = other DNA
accacgtacaccagg

SEQ ID NO: 379 - DNA, 15 bp, synthetic construct
  misc_feature 1..15: note = >DNA sequence encoding for cyclic peptide C5-385
  source 1..15: mol_type = other DNA
accacgctgtaccgg

SEQ ID NO: 380 - DNA, 15 bp, synthetic construct
  misc_feature 1..15: note = >DNA sequence encoding for cyclic peptide C5-389
  source 1..15: mol_type = other DNA
acccacctggaccgg

SEQ ID NO: 381 - DNA, 15 bp, synthetic construct
  misc_feature 1..15: note = >DNA sequence encoding for cyclic peptide C5-391
  source 1..15: mol_type = other DNA
accttgttgatcagg

SEQ ID NO: 382 - DNA, 15 bp, synthetic construct
  misc_feature 1..15: note = >DNA sequence encoding for cyclic peptide C5-392
  source 1..15: mol_type = other DNA
accacgtgcgaccgg

SEQ ID NO: 383 - DNA, 15 bp, synthetic construct
  misc_feature 1..15: note = >DNA sequence encoding for cyclic peptide C5-393
  source 1..15: mol_type = other DNA
accacgggtcgccgg

SEQ ID NO: 384 - DNA, 15 bp, synthetic construct
  misc_feature 1..15: note = >DNA sequence encoding for cyclic peptide C5-394
  source 1..15: mol_type = other DNA
accaccgtgagccgg

SEQ ID NO: 385 - DNA, 15 bp, synthetic construct
  misc_feature 1..15: note = >DNA sequence encoding for cyclic peptide C5-395
  source 1..15: mol_type = other DNA
accacgcagcaccgg

SEQ ID NO: 386 - DNA, 15 bp, synthetic construct
  misc_feature 1..15: note = >DNA sequence encoding for cyclic peptide C5-396
  source 1..15: mol_type = other DNA
accactacgcccagg

SEQ ID NO: 387 - DNA, 15 bp, synthetic construct
  misc_feature 1..15: note = >DNA sequence encoding for cyclic peptide C5-399
  source 1..15: mol_type = other DNA
accgccttcgcccgg

SEQ ID NO: 388 - DNA, 15 bp, synthetic construct
  misc_feature 1..15: note = >DNA sequence encoding for cyclic peptide C5-405
  source 1..15: mol_type = other DNA
accacgtcacaccgg

SEQ ID NO: 389 - DNA, 15 bp, synthetic construct
  misc_feature 1..15: note = >DNA sequence encoding for cyclic peptide C5-410
  source 1..15: mol_type = other DNA
accgtcttgggccgg

SEQ ID NO: 390 - DNA, 15 bp, synthetic construct
  misc_feature 1..15: note = >DNA sequence encoding for cyclic peptide C5-411
  source 1..15: mol_type = other DNA
accacgcagcgcagg

SEQ ID NO: 391 - DNA, 15 bp, synthetic construct
  misc_feature 1..15: note = >DNA sequence encoding for cyclic peptide C5-413
  source 1..15: mol_type = other DNA
accagtcacgccagg

SEQ ID NO: 392 - DNA, 15 bp, synthetic construct
  misc_feature 1..15: note = >DNA sequence encoding for cyclic peptide C5-415
  source 1..15: mol_type = other DNA
accacgacgtgccgg

SEQ ID NO: 393 - DNA, 15 bp, synthetic construct
  misc_feature 1..15: note = >DNA sequence encoding for cyclic peptide C5-422
  source 1..15: mol_type = other DNA
accgcgtggcgccgc

SEQ ID NO: 394 - DNA, 15 bp, synthetic construct
  misc_feature 1..15: note = >DNA sequence encoding for cyclic peptide C5-428
  source 1..15: mol_type = other DNA
accacgtgtggccgg

SEQ ID NO: 395 - DNA, 15 bp, synthetic construct
  misc_feature 1..15: note = >DNA sequence encoding for cyclic peptide C5-434
  source 1..15: mol_type = other DNA
accacctctggccgg

SEQ ID NO: 396 - DNA, 15 bp, synthetic construct
  misc_feature 1..15: note = >DNA sequence encoding for cyclic peptide C5-438
  source 1..15: mol_type = other DNA
accacgacgtcgagg

SEQ ID NO: 397 - DNA, 15 bp, synthetic construct
  misc_feature 1..15: note = >DNA sequence encoding for cyclic peptide C5-440
  source 1..15: mol_type = other DNA
accgcgactggacgg

SEQ ID NO: 398 - DNA, 15 bp, synthetic construct
  misc_feature 1..15: note = >DNA sequence encoding for cyclic peptide C5-441
  source 1..15: mol_type = other DNA
accgcgtgggaccgg

SEQ ID NO: 399 - DNA, 15 bp, synthetic construct
  misc_feature 1..15: note = >DNA sequence encoding for cyclic peptide C5-443
  source 1..15: mol_type = other DNA
accacgcatcaccgg

SEQ ID NO: 400 - DNA, 15 bp, synthetic construct
  misc_feature 1..15: note = >DNA sequence encoding for cyclic peptide C5-448
  source 1..15: mol_type = other DNA
accgcgtacgccagg

SEQ ID NO: 401 - DNA, 15 bp, synthetic construct
  misc_feature 1..15: note = >DNA sequence encoding for cyclic peptide C5-449
  source 1..15: mol_type = other DNA
accgcgaacgcgagg

SEQ ID NO: 402 - DNA, 15 bp, synthetic construct
  misc_feature 1..15: note = >DNA sequence encoding for cyclic peptide C5-450
  source 1..15: mol_type = other DNA
acccgcgacgtgagg

SEQ ID NO: 403 - DNA, 15 bp, synthetic construct
  misc_feature 1..15: note = >DNA sequence encoding for cyclic peptide C5-452
  source 1..15: mol_type = other DNA
acccacgtcgacagg

SEQ ID NO: 404 - DNA, 15 bp, synthetic construct
  misc_feature 1..15: note = >DNA sequence encoding for cyclic peptide C5-453
  source 1..15: mol_type = other DNA
accctattctggcgg

SEQ ID NO: 405 - DNA, 15 bp, synthetic construct
  misc_feature 1..15: note = >DNA sequence encoding for cyclic peptide C5-459
  source 1..15: mol_type = other DNA
accaccgcggcccgg

SEQ ID NO: 406 - DNA, 15 bp, synthetic construct
  misc_feature 1..15: note = >DNA sequence encoding for cyclic peptide C5-463
  source 1..15: mol_type = other DNA
accgtcgtggaccgg

SEQ ID NO: 407 - DNA, 15 bp, synthetic construct
  misc_feature 1..15: note = >DNA sequence encoding for cyclic peptide C5-464
  source 1..15: mol_type = other DNA
accactccggcccgg

SEQ ID NO: 408 - DNA, 15 bp, synthetic construct
  misc_feature 1..15: note = >DNA sequence encoding for cyclic peptide C5-469
  source 1..15: mol_type = other DNA
accacgatcggcagg

SEQ ID NO: 409 - DNA, 15 bp, synthetic construct
  misc_feature 1..15: note = >DNA sequence encoding for cyclic peptide C5-472
  source 1..15: mol_type = other DNA
accatgtacgccagg

SEQ ID NO: 410 - DNA, 15 bp, synthetic construct
  misc_feature 1..15: note = >DNA sequence encoding for cyclic peptide C5-473
  source 1..15: mol_type = other DNA
acccacgtggccagg

SEQ ID NO: 411 - DNA, 15 bp, synthetic construct
  misc_feature 1..15: note = >DNA sequence encoding for cyclic peptide C5-474
  source 1..15: mol_type = other DNA
accacctggccgcgg

SEQ ID NO: 412 - DNA, 15 bp, synthetic construct
  misc_feature 1..15: note = >DNA sequence encoding for cyclic peptide C5-475
  source 1..15: mol_type = other DNA
accaccggtgaccgg

SEQ ID NO: 413 - DNA, 15 bp, synthetic construct
  misc_feature 1..15: note = >DNA sequence encoding for cyclic peptide C5-479
  source 1..15: mol_type = other DNA
accacgaccgtgcgg

SEQ ID NO: 414 - DNA, 15 bp, synthetic construct
  misc_feature 1..15: note = >DNA sequence encoding for cyclic peptide C5-481
  source 1..15: mol_type = other DNA
accgtctttggcagg

SEQ ID NO: 415 - DNA, 15 bp, synthetic construct
  misc_feature 1..15: note = >DNA sequence encoding for cyclic peptide C5-483
  source 1..15: mol_type = other DNA
acccgtgtgggccgg

SEQ ID NO: 416 - DNA, 18 bp, synthetic construct
  misc_feature 1..18: note = >DNA sequence encoding for cyclic peptide A C6-1
  source 1..18: mol_type = other DNA
accccggtctggttcgac

SEQ ID NO: 417 - DNA, 18 bp, synthetic construct
  misc_feature 1..18: note = >DNA sequence encoding for cyclic peptide A C6-2
  source 1..18: mol_type = other DNA
accccggcctggttcgac

SEQ ID NO: 418 - DNA, 18 bp, synthetic construct
  misc_feature 1..18: note = >DNA sequence encoding for cyclic peptide A C6-4
  source 1..18: mol_type = other DNA
accttggagttcttcgac

SEQ ID NO: 419 - DNA, 18 bp, synthetic construct
  misc_feature 1..18: note = >DNA sequence encoding for cyclic peptide A C6-6
  source 1..18: mol_type = other DNA
accgtcacgtggttcgac

SEQ ID NO: 420 - DNA, 18 bp, synthetic construct
  misc_feature 1..18: note = >DNA sequence encoding for cyclic peptide A C6-8
  source 1..18: mol_type = other DNA
accttgttgatcaggtgg

SEQ ID NO: 421 - DNA, 18 bp, synthetic construct
  misc_feature 1..18: note = >DNA sequence encoding for cyclic peptide A C6-10
  source 1..18: mol_type = other DNA
accctcaagtggctgaac

SEQ ID NO: 422 - DNA, 18 bp, synthetic construct
  misc_feature 1..18: note = >DNA sequence encoding for cyclic peptide A C6-21
  source 1..18: mol_type = other DNA
accaaggagtacttcgac

SEQ ID NO: 423 - DNA, 18 bp, synthetic construct
  misc_feature 1..18: note = >DNA sequence encoding for cyclic peptide A C6-26
  source 1..18: mol_type = other DNA
accctccactggttcgag

SEQ ID NO: 424 - DNA, 18 bp, synthetic construct
  misc_feature 1..18: note = >DNA sequence encoding for cyclic peptide A C6-27
  source 1..18: mol_type = other DNA
acctgctcgtggttcgac

SEQ ID NO: 425 - DNA, 18 bp, synthetic construct
  misc_feature 1..18: note = >DNA sequence encoding for cyclic peptide A C6-28
  source 1..18: mol_type = other DNA
accctcgagtacttcatg

SEQ ID NO: 426 - DNA, 18 bp, synthetic construct
  misc_feature 1..18: note = >DNA sequence encoding for cyclic peptide A C6-32
  source 1..18: mol_type = other DNA
accctgtgctggctcaac

SEQ ID NO: 427 - DNA, 18 bp, synthetic construct
  misc_feature 1..18: note = >DNA sequence encoding for cyclic peptide A C6-36
  source 1..18: mol_type = other DNA
accccgatcgtgttcgac

SEQ ID NO: 428 - DNA, 18 bp, synthetic construct
  misc_feature 1..18: note = >DNA sequence encoding for cyclic peptide A C6-37
  source 1..18: mol_type = other DNA
accctgtgggtcttcgac

SEQ ID NO: 429 - DNA, 18 bp, synthetic construct
  misc_feature 1..18: note = >DNA sequence encoding for cyclic peptide A C6-40
  source 1..18: mol_type = other DNA
acccccttgtggttcaac

SEQ ID NO: 430 - DNA, 18 bp, synthetic construct
  misc_feature 1..18: note = >DNA sequence encoding for cyclic peptide A C6-41
  source 1..18: mol_type = other DNA
acctcggtcgagtacgag

SEQ ID NO: 431 - DNA, 18 bp, synthetic construct
  misc_feature 1..18: note = >DNA sequence encoding for cyclic peptide A C6-42
  source 1..18: mol_type = other DNA
accctgggctggttggac

SEQ ID NO: 432 - DNA, 18 bp, synthetic construct
  misc_feature 1..18: note = >DNA sequence encoding for cyclic peptide A C6-44
  source 1..18: mol_type = other DNA
accccgccctggttcgac

SEQ ID NO: 433 - DNA, 18 bp, synthetic construct
  misc_feature 1..18: note = >DNA sequence encoding for cyclic peptide A C6-46
  source 1..18: mol_type = other DNA
accccgtgctggttcgac

SEQ ID NO: 434 - DNA, 18 bp, synthetic construct
  misc_feature 1..18: note = >DNA sequence encoding for cyclic peptide A C6-47
  source 1..18: mol_type = other DNA
accttgtcctggtacgac

SEQ ID NO: 435 - DNA, 18 bp, synthetic construct
  misc_feature 1..18: note = >DNA sequence encoding for cyclic peptide A C6-48
  source 1..18: mol_type = other DNA
accccggtcctggtcgac

SEQ ID NO: 436 - DNA, 18 bp, synthetic construct
  misc_feature 1..18: note = >DNA sequence encoding for cyclic peptide A C6-49
  source 1..18: mol_type = other DNA
accctcgagtacttgtgg

SEQ ID NO: 437 - DNA, 18 bp, synthetic construct
  misc_feature 1..18: note = >DNA sequence encoding for cyclic peptide A C6-50
  source 1..18: mol_type = other DNA
accatcttctggttcgac

SEQ ID NO: 438 - DNA, 18 bp, synthetic construct
  misc_feature 1..18: note = >DNA sequence encoding for cyclic peptide A C6-53
  source 1..18: mol_type = other DNA
accccggccctggtcgac

SEQ ID NO: 439 - DNA, 18 bp, synthetic construct
  misc_feature 1..18: note = >DNA sequence encoding for cyclic peptide A C6-55
  source 1..18: mol_type = other DNA
acccccggctggttcgac

SEQ ID NO: 440 - DNA, 18 bp, synthetic construct
  misc_feature 1..18: note = >DNA sequence encoding for cyclic peptide A C6-57
  source 1..18: mol_type = other DNA
accttgtccgtcttcgac

SEQ ID NO: 441 - DNA, 18 bp, synthetic construct
  misc_feature 1..18: note = >DNA sequence encoding for cyclic peptide A C6-58
  source 1..18: mol_type = other DNA
acccccggtctggtcgac

SEQ ID NO: 442 - DNA, 18 bp, synthetic construct
  misc_feature 1..18: note = >DNA sequence encoding for cyclic peptide A C6-59
  source 1..18: mol_type = other DNA
accctctcctggttcaac

SEQ ID NO: 443 - DNA, 18 bp, synthetic construct
  misc_feature 1..18: note = >DNA sequence encoding for cyclic peptide A C6-63
  source 1..18: mol_type = other DNA
accttggacttcttcgac

SEQ ID NO: 444 - DNA, 18 bp, synthetic construct
  misc_feature 1..18: note = >DNA sequence encoding for cyclic peptide A C6-65
  source 1..18: mol_type = other DNA
accccgtcctggttcgac

SEQ ID NO: 445 - DNA, 18 bp, synthetic construct
  misc_feature 1..18: note = >DNA sequence encoding for cyclic peptide A C6-68
  source 1..18: mol_type = other DNA
accccggccctgttcgac

SEQ ID NO: 446 - DNA, 18 bp, synthetic construct
  misc_feature 1..18: note = >DNA sequence encoding for cyclic peptide A C6-69
  source 1..18: mol_type = other DNA
accccggcctggtccgac

SEQ ID NO: 447 - DNA, 18 bp, synthetic construct
  misc_feature 1..18: note = >DNA sequence encoding for cyclic peptide A C6-78
  source 1..18: mol_type = other DNA
accccggcccggttcgac

SEQ ID NO: 448 - DNA, 18 bp, synthetic construct
  misc_feature 1..18: note = >DNA sequence encoding for cyclic peptide A C6-79
  source 1..18: mol_type = other DNA
accccggcctggctcgac

SEQ ID NO: 449 - DNA, 18 bp, synthetic construct
  misc_feature 1..18: note = >DNA sequence encoding for cyclic peptide A C6-80
  source 1..18: mol_type = other DNA
accccggtctggctcgac

SEQ ID NO: 450 - DNA, 12 bp, synthetic construct
  misc_feature 1..12: note = >DNA sequence encoding for cyclic peptide C4-9
  source 1..12: mol_type = other DNA
accacgtgccgg

SEQ ID NO: 451 - DNA, 12 bp, synthetic construct
  misc_feature 1..12: note = >DNA sequence encoding for cyclic peptide C4-11
  source 1..12: mol_type = other DNA
accactcgccgg

SEQ ID NO: 452 - DNA, 12 bp, synthetic construct
  misc_feature 1..12: note = >DNA sequence encoding for cyclic peptide C4-31
  source 1..12: mol_type = other DNA
accacgtcgcgg

SEQ ID NO: 453 - DNA, 12 bp, synthetic construct
  misc_feature 1..12: note = >DNA sequence encoding for cyclic peptide C4-34
  source 1..12: mol_type = other DNA
acacgtggacgg

SEQ ID NO: 454 - DNA, 12 bp, synthetic construct
  misc_feature 1..12: note = >DNA sequence encoding for cyclic peptide C4-35
  source 1..12: mol_type = other DNA
accactggccgg

SEQ ID NO: 455 - DNA, 12 bp, synthetic construct
  misc_feature 1..12: note = >DNA sequence encoding for cyclic peptide C4-41
  source 1..12: mol_type = other DNA
acacgtcgcagg

SEQ ID NO: 456 - DNA, 12 bp, synthetic construct
  misc_feature 1..12: note = >DNA sequence encoding for cyclic peptide A C4B-9
  source 1..12: mol_type = other DNA
accgaccagcgg

SEQ ID NO: 457 - DNA, 12 bp, synthetic construct
  misc_feature 1..12: note = >DNA sequence encoding for cyclic peptide A C4B-41
  source 1..12: mol_type = other DNA
accctgatccgc

SEQ ID NO: 458 - DNA, 12 bp, synthetic construct
  misc_feature 1..12: note = >DNA sequence encoding for cyclic peptide A C4B-80
  source 1..12: mol_type = other DNA
accctgtggcgg

SEQ ID NO: 459 - DNA, 12 bp, synthetic construct
  misc_feature 1..12: note = >DNA sequence encoding for cyclic peptide A C4B-86
  source 1..12: mol_type = other DNA
accttgggccgg

SEQ ID NO: 460 - DNA, 12 bp, synthetic construct
  misc_feature 1..12: note = >DNA sequence encoding for cyclic peptide C5( 2)
  source 1..12: mol_type = other DNA
accttcgaccgg

SEQ ID NO: 461 - DNA, 12 bp, synthetic construct
  misc_feature 1..12: note = >DNA sequence encoding for cyclic peptide C5( D4)
  source 1..12: mol_type = other DNA
accgcgttccgg

SEQ ID NO: 462 - DNA, 15 bp, synthetic construct
  misc_feature 1..15: note = >DNA sequence encoding for cyclic peptide SOD1C5-1
  source 1..15: mol_type = other DNA
accgcctcgtggtgg

SEQ ID NO: 463 - DNA, 15 bp, synthetic construct
  misc_feature 1..15: note = >DNA sequence encoding for cyclic peptide SOD1C5-2
  source 1..15: mol_type = other DNA
accgcgagcttctgg

SEQ ID NO: 464 - DNA, 15 bp, synthetic construct
  misc_feature 1..15: note = >DNA sequence encoding for cyclic peptide SOD1C5-3
  source 1..15: mol_type = other DNA
acctcgtcgttctgg

SEQ ID NO: 465 - DNA, 15 bp, synthetic construct
  misc_feature 1..15: note = >DNA sequence encoding for cyclic peptide SOD1C5-4
  source 1..15: mol_type = other DNA
acctggtccgtgtgg

SEQ ID NO: 466 - DNA, 15 bp, synthetic construct
  misc_feature 1..15: note = >DNA sequence encoding for cyclic peptide SOD1C5-5
  source 1..15: mol_type = other DNA
accgccagccactgg

SEQ ID NO: 467 - DNA, 15 bp, synthetic construct
  misc_feature 1..15: note = >DNA sequence encoding for cyclic peptide SOD1C5-6
  source 1..15: mol_type = other DNA
accttcagcatgtgg

SEQ ID NO: 468 - DNA, 15 bp, synthetic construct
  misc_feature 1..15: note = >DNA sequence encoding for cyclic peptide SOD1C5-7
  source 1..15: mol_type = other DNA
accgcctcgatgtgg

SEQ ID NO: 469 - DNA, 15 bp, synthetic construct
  misc_feature 1..15: note = >DNA sequence encoding for cyclic peptide SOD1C5-9
  source 1..15: mol_type = other DNA
accgtctcgttctgg

SEQ ID NO: 470 - DNA, 15 bp, synthetic construct
  misc_feature 1..15: note = >DNA sequence encoding for cyclic peptide SOD1C5-11
  source 1..15: mol_type = other DNA
accctctccttctgg

SEQ ID NO: 471 - DNA, 15 bp, synthetic construct
  misc_feature 1..15: note = >DNA sequence encoding for cyclic peptide SOD1C5-13
  source 1..15: mol_type = other DNA
accgccagccgctgg

SEQ ID NO: 472 - DNA, 15 bp, synthetic construct
  misc_feature 1..15: note = >DNA sequence encoding for cyclic peptide SOD1C5-14
  source 1..15: mol_type = other DNA
accgcgagctcgtgg

SEQ ID NO: 473 - DNA, 15 bp, synthetic construct
  misc_feature 1..15: note = >DNA sequence encoding for cyclic peptide SOD1C5-18
  source 1..15: mol_type = other DNA
accgcgagcctctgg

SEQ ID NO: 474 - DNA, 15 bp, synthetic construct
  misc_feature 1..15: note = >DNA sequence encoding for cyclic peptide SOD1C5-20
  source 1..15: mol_type = other DNA
acctcgtcgtcctgg

SEQ ID NO: 475 - DNA, 15 bp, synthetic construct
  misc_feature 1..15: note = >DNA sequence encoding for cyclic peptide SOD1C5-23
  source 1..15: mol_type = other DNA
accggctccgtgtgg

SEQ ID NO: 476 - DNA, 15 bp, synthetic construct
  misc_feature 1..15: note = >DNA sequence encoding for cyclic peptide SOD1C5-25
  source 1..15: mol_type = other DNA
acctggtccctgtgg

SEQ ID NO: 477 - DNA, 15 bp, synthetic construct
  misc_feature 1..15: note = >DNA sequence encoding for cyclic peptide SOD1C5-27
  source 1..15: mol_type = other DNA
accctcagcatgtgg

SEQ ID NO: 478 - DNA, 15 bp, synthetic construct
  misc_feature 1..15: note = >DNA sequence encoding for cyclic peptide SOD1C5-31
  source 1..15: mol_type = other DNA
acctggtccgcgtgg

SEQ ID NO: 479 - DNA, 15 bp, synthetic construct
  misc_feature 1..15: note = >DNA sequence encoding for cyclic peptide SOD1C5-32
  source 1..15: mol_type = other DNA
accggctcgtggtgg

SEQ ID NO: 480 - DNA, 15 bp, synthetic construct
  misc_feature 1..15: note = >DNA sequence encoding for cyclic peptide SOD1C5-33
  source 1..15: mol_type = other DNA
acccggtccgtgtgg

SEQ ID NO: 481 - DNA, 15 bp, synthetic construct
  misc_feature 1..15: note = >DNA sequence encoding for cyclic peptide SOD1C5-39
  source 1..15: mol_type = other DNA
acctcgtcgctctgg

SEQ ID NO: 482 - DNA, 15 bp, synthetic construct
  misc_feature 1..15: note = >DNA sequence encoding for cyclic peptide SOD1C5-44
  source 1..15: mol_type = other DNA
accgccagcacctgg

SEQ ID NO: 483 - DNA, 15 bp, synthetic construct
  misc_feature 1..15: note = >DNA sequence encoding for cyclic peptide SOD1C5-46
  source 1..15: mol_type = other DNA
acctcgtccgtctgg

SEQ ID NO: 484 - DNA, 15 bp, synthetic construct
  misc_feature 1..15: note = >DNA sequence encoding for cyclic peptide SOD1C5-53
  source 1..15: mol_type = other DNA
accacctcgtggtgg

SEQ ID NO: 485 - DNA, 15 bp, synthetic construct
  misc_feature 1..15: note = >DNA sequence encoding for cyclic peptide SOD1C5-65
  source 1..15: mol_type = other DNA
accgcgagcgtctgg

SEQ ID NO: 486 - DNA, 15 bp, synthetic construct
  misc_feature 1..15: note = >DNA sequence encoding for cyclic peptide SOD1C5-74
  source 1..15: mol_type = other DNA
acctgctcgtggtgg

SEQ ID NO: 487 - DNA, 15 bp, synthetic construct
  misc_feature 1..15: note = >DNA sequence encoding for cyclic peptide SOD1C5-75
  source 1..15: mol_type = other DNA
accccgtcgttctgg

SEQ ID NO: 488 - DNA, 15 bp, synthetic construct
  misc_feature 1..15: note = >DNA sequence encoding for cyclic peptide SOD1C5-76
  source 1..15: mol_type = other DNA
accacgagcttctgg

SEQ ID NO: 489 - DNA, 15 bp, synthetic construct
  misc_feature 1..15: note = >DNA sequence encoding for cyclic peptide SOD1C5-80
  source 1..15: mol_type = other DNA
accttcagcacgtgg

SEQ ID NO: 490 - DNA, 15 bp, synthetic construct
  misc_feature 1..15: note = >DNA sequence encoding for cyclic peptide SOD1C5-82
  source 1..15: mol_type = other DNA
acctcgagcatgtgg

SEQ ID NO: 491 - DNA, 15 bp, synthetic construct
  misc_feature 1..15: note = >DNA sequence encoding for cyclic peptide SOD1C5-89
  source 1..15: mol_type = other DNA
accgtctcgtggtgg

SEQ ID NO: 492 - DNA, 15 bp, synthetic construct
  misc_feature 1..15: note = >DNA sequence encoding for cyclic peptide SOD1C5-93
  source 1..15: mol_type = other DNA
accgactcgtggtgg

SEQ ID NO: 493 - DNA, 15 bp, synthetic construct
  misc_feature 1..15: note = >DNA sequence encoding for cyclic peptide SOD1C5-105
  source 1..15: mol_type = other DNA
acctcgtcctggtgg

SEQ ID NO: 494 - DNA, 15 bp, synthetic construct
  misc_feature 1..15: note = >DNA sequence encoding for cyclic peptide SOD1C5-106
  source 1..15: mol_type = other DNA
acccgctcgtggtgg

SEQ ID NO: 495 - DNA, 15 bp, synthetic construct
  misc_feature 1..15: note = >DNA sequence encoding for cyclic peptide SOD1C5-109
  source 1..15: mol_type = other DNA
acctggtccatgtgg

SEQ ID NO: 496 - DNA, 15 bp, synthetic construct
  misc_feature 1..15: note = >DNA sequence encoding for cyclic peptide SOD1C5-116
  source 1..15: mol_type = other DNA
accgcctctgggtgg

SEQ ID NO: 497 - DNA, 15 bp, synthetic construct
  misc_feature 1..15: note = >DNA sequence encoding for cyclic peptide SOD1C5-130
  source 1..15: mol_type = other DNA
acgccctcgtggtgg

SEQ ID NO: 498 - DNA, 15 bp, synthetic construct
  misc_feature 1..15: note = >DNA sequence encoding for cyclic peptide SOD1C5-135
  source 1..15: mol_type = other DNA
acgcggagcttctgg

SEQ ID NO: 499 - DNA, 15 bp, synthetic construct
  misc_feature 1..15: note = >DNA sequence encoding for cyclic peptide SOD1C5-140
  source 1..15: mol_type = other DNA
acctcgtcctactgg

SEQ ID NO: 500 - DNA, 15 bp, synthetic construct
  misc_feature 1..15: note = >DNA sequence encoding for cyclic peptide SOD1C5-143
  source 1..15: mol_type = other DNA
accttgagcgtgtgg

SEQ ID NO: 501 - DNA, 15 bp, synthetic construct
  misc_feature 1..15: note = >DNA sequence encoding for cyclic peptide SOD1C5-148
  source 1..15: mol_type = other DNA
acctactcatggtgg

SEQ ID NO: 502 - DNA, 15 bp, synthetic construct
  misc_feature 1..15: note = >DNA sequence encoding for cyclic peptide SOD1C5-160
  source 1..15: mol_type = other DNA
accttcagcgtgtgg

SEQ ID NO: 503 - DNA, 15 bp, synthetic construct
  misc_feature 1..15: note = >DNA sequence encoding for cyclic peptide SOD1C5-164
  source 1..15: mol_type = other DNA
acctgcttcgtgtgg

SEQ ID NO: 504 - DNA, 15 bp, synthetic construct
  misc_feature 1..15: note = >DNA sequence encoding for cyclic peptide SOD1C5-167
  source 1..15: mol_type = other DNA
accgtctcgtcgtgg

SEQ ID NO: 505 - DNA, 15 bp, synthetic construct
  misc_feature 1..15: note = >DNA sequence encoding for cyclic peptide SOD1C5-168
  source 1..15: mol_type = other DNA
acccgcagccactgg

SEQ ID NO: 506 - DNA, 15 bp, synthetic construct
  misc_feature 1..15: note = >DNA sequence encoding for cyclic peptide SOD1C5-182
  source 1..15: mol_type = other DNA
accggcagcgcgtgg

SEQ ID NO: 507 - DNA, 15 bp, synthetic construct
  misc_feature 1..15: note = >DNA sequence encoding for cyclic peptide SOD1C5-188
  source 1..15: mol_type = other DNA
accgccagctactgg

SEQ ID NO: 508 - protein, 8 aa, synthetic construct
  VARIANT 7..8: note = X can be any amino acid
AIGHNCXX

SEQ ID NO: 509 - protein, 8 aa, synthetic construct
  VARIANT 7..8: note = X can be any amino acid
AIGHNSXX

SEQ ID NO: 510 - protein, 8 aa, synthetic construct
  VARIANT 7..8: note = X can be any amino acid
AIGHNTXX

SEQ ID NO: 511 - protein, 6 aa, synthetic construct
  VARIANT 1: note = X can be any amino acid
XCLSFG

SEQ ID NO: 512 - DNA, 24 bp, unidentified
  source 1..24: mol_type = other DNA
  variation 19..20: note = n can be a or c or g or t/u
  variation 22..23: note = n can be a or c or g or t/u
  variation 21: note = s can be c or g
  variation 24: note = s can be c or g
gcgatcggccacaattgcnnsnns

SEQ ID NO: 513 - DNA, 24 bp, synthetic construct
  source 1..24: mol_type = other DNA
  variation 19..20: note = n can be a or c or g or t/u
  variation 22..23: note = n can be a or c or g or t/u
  variation 21: note = s can be c or g
  variation 24: note = s can be c or g
gcgatcggccacaatagcnnsnns

SEQ ID NO: 514 - DNA, 24 bp, synthetic construct
  source 1..24: mol_type = other DNA
  variation 19..20: note = n can be a or c or g or t/u
  variation 22..23: note = n can be a or c or g or t/u
  variation 21: note = s can be c or g
  variation 24: note = s can be c or g
gcgatcggccacaataccnnsnns

SEQ ID NO: 515 - DNA, 18 bp, synthetic construct
  source 1..18: mol_type = other DNA
  variation 1..2: note = n can be a or c or g or t/u
  variation 3: note = s can be c or g
nnstgcttaagttttggc